European Patent Specification EP 3 916 111 B1, published August 9, 2023. Title: Universal Primer Sets for Detecting Flavivirus and Use Thereof. Applicant: INDUSTRY FOUNDATION OF CHONNAM NATIONAL UNIVERSITY. The sequence listing filed with the application follows.

SEQUENCE LISTING (16 sequences)

SEQ ID NO: 1 - DNA, 29 bp, Artificial Sequence
  L2CNU3-F_Pflavi
tacaacatgatgggvaaragagaraaraa

SEQ ID NO: 2 - DNA, 22 bp, Artificial Sequence
  L2CNU3-R5_Pflavi
ccrgcrgtrtcatcrgcrtasa

SEQ ID NO: 3 - DNA, 10706 bp, Artificial Sequence
  DENV1_ MF314188
tctacgtggaccgacaagaacagtttcgaatcggaagcttgcttaacgtagttctgacagttttttattagagagcagatctctgatgaacaaccaacgaaaaaagacggctcgaccgtctttcaatatgctgaaacgcgcgagaaaccgcgtgtcaactgtttcacagttggcgaagagattctcaaaaggattgctctcaggccaaggacccatgaaactggtgatggctttcatagcattcctaagatttctagccatacccccaacagcaggaattttggctagatggggctcattcaagaagaatggagcgatcaaagtgctacggggtttcaagaaagaaatctcaagcatgttgaatataatgaatagaaggaaaagatctgtgaccatgctccttatgctgatgcctacagccttggcattccatttgactacacgagggggagagccgcacatgatagtcagcaagcaggaaagaggaaagtcacttttgtttaagacctcagcaggtgtcaacatgtgcaccctcatagcgatggatttgggagagttatgtgaggacacaatgacttacaaatgccctcgaatcactgaggcggaaccagatgacgttgattgttggtgcaatgccacaaacacatgggtgacctatggaacatgttcccaaactggcgagcaccgacgagacaaacgttccgttgcactggccccacacgtgggacttggtttggaaacaagaaccgaaacgtggatgtcctctgaaggcgcttggaaacagatacaaagagtggagacttgggccctgagacacccaggattcacggtgatagccctttttctagcacatgccataggaacatccatcacccagaaagggattatcttcattttgttaatgctggttacaccatctatggccatgcgatgcgtgggaataggcagcagggacttcgtggaaggactgtcaggagcaacttgggtagatgtggtgttggaacatggaagttgcgtcactaccatggcaaaagacaaaccaacattggacattgaactcttgaagacggaagtcacaaaccctgccgtcctgcgcaaactgtgcattgaagctaaaatatcaaacaccaccaccgactcaagatgtccaacacaaggagaagccacactggtggaagaacaagacgcgaactttgtgtgtcgacgaacgtttgtggacagaggctggggcaatggatgtgggctcttcggaaaaggaagccttataacgtgtgccaagttcaagtgtgtgacaaaactggaaggaaaaatagttcaatatgaaaacttgaaatattcagtaatagtcaccgtccacactggagaccagcaccaggtgggaaatgaaagcacagaacatgggacaactgcaaccataacacctcaagctcctacgacagaaatacagctgaccgactacggagctcttacattggattgttcacctagaacaggactggacttcaatgaaatggtgttgttgacaatgaaagaaaaatcatggctagtccacaaacaatggtttctagacctaccattgccttggacctcgggagcttcaacatcacaagaaacttggaacagacaagatttgctggtgacatttaagacagctcatgcaaagaagcaggaagtagtcgtactaggatcacaagaaggagcaatgcacactgcgttgaccggagcgacggaaatccaaacgtctggaacgacaacaatttttgcaggacacttgaaatgtagactaaagatggacaaactgactctaaaagggatgtcatatgtgatgtgcacaggctcattcaagctagagaaagaaatggctgagacccagcatggaaccgttctagtgcagattaaatacgaaggaacagatgcaccatgcaagatccctttttcgacccaagatgaaaaaggagtaacccagaatgggagattgataacagccaaccccatagtcactgacaaagaaaaaccagtcaacattgaggcagaaccgccttttggtgagagttacatcgtgataggagcaggtgaaaaggctttgaaactaagctggttcaagaaaggaagcagcatagggaaaatgtttgaggcaactgccagaggagcacgaaggatggccatactgggagacaccgcatgggactttggttctataggaggagtgttcacgtctgttggaaaattagtacaccagatttttggaactgcatatggagttttgttcagcggtgtttcctggaccatgaaaataggaataggggttctgctgacatggctaggattaaactcaaggagcacgtccctttcgatgacgtgcattgcagtcggcctagtaacgctatacttaggagtcatggttcaggcggattcaggatgtgtaattaattggaaaggtagagaactcaaatgtgggagtggcatttttgtcactaatgaagttcacacttggacagagcaatacaaatttcaagctgattccccaaagagactatcagcagccattgggaaggcatgggaggagggtgtgtgtggaattcgatcagcaacccgtctcgagaacatcatgtggaagcaaatatcaaatgaattgaaccacatcttgcttgaaaatgacatgaaattcacagtggttgtaggagatgttgctgggatcttggctcaaggaaaaaaaatgattaggccacaacccatggaacacaaatactcgtggaaaagctggggaaaagctaaaatcataggggcagatgtacagaacaccacctttatcatcgacggcccaaacaccccagaatgccctgatgatcaaagagcatggaacatttgggaagttgaggattatggatttggaattttcacgacaaacatatggctgaaattgcgtgactcctacacccaagtgtgtgaccaccggctaatgtcagctgccatcaaagacagcaaggcagttcatgctgacatggggtactggatagaaagtgaaaagaacgagacctggaagctggcaagagcctctttcatagaagtcaaaacgtgtatctggccaaaatctcacactctatggagcaacggagttctggaaagtgaaatgataattccaaagatctatggaggaccaatatctcagcacaactacagaccaggatatttcacacaaacggcagggccgtggcatctaggcaagttggaactggattttgatttgtgtgagggtaccacggttgttgtggatgaacattgtggaaatcgaggaccatctcttaggaccacaacagtcacaggaaagataattcatgaatggtgttgcagatcttgtacgctaccacccttacgtttcagaggagaagatgggtgctggtacggtatggaaatcagaccagtcaaggagaaggaagagaatctagtcaaatcaatggtctctgcagggttaggggaagtggacagcttttcactaggactgttatgcatatcaataatgatcgaagaggtgatgagatccagatggagtagaaaaatgctgatgactggaacactggctgtgttcttccttctcataatgggacaattgacatggaatgatctgatcagattatgcatcatggttggagccaacgcttccgacaggatggggatgggaacgacctacctagctctgatggccacttttaaaatgagaccaatgtttgccgtagggctactattccgcagactaacatccagagaagttcttcttctaacaattggattgagtctagtggcatctgtggagttaccaaattccttggaggagctgggggatggacttgcaatgggcattatgatcttaaaattattgactgactttcaatcacatcagctgtgggctaccttgctgtccttgacatttatcaaaacaacgttttccttgcactatgcatggaagacaatggctatggtactgtcaattgtatctctcttccccttatgcctgtccacgacctcccaaaaaacaacatggcttccggtgctgttgggatctcttggatgcaaaccactaaccatgtttcttatagcagaaaacaaaatctgggggaggaaaagttggcccctcaatgaaggaatcatggctgttggaatagtcagcatcctactaagttcactcctcaaaaatgatgtgccgctagctgggccattgatagctggaggcatgctaatagcatgttatgtcatatctggaagctcagccgatctatcactagagaaagcggctgaggtctcctgggaagaagaagcagaacactctggtgcctcacacaacatattagtggaggtccaagatgatggaaccatgaagataaaggatgaagagagagatgacacgctaaccattctccttaaagcaactctgctagcaatttcaggggtgtacccattatcaataccagcgacccttcttgtgtggtacttttggcagaaaaagaaacagagatctggagtgttatgggacacacctagccctccagaagtggaaagagcagttcttgatgatggcatctatagaatcatgcagagaggactgttgggcaggtcccaagtgggggtaggagtgtttcaagaaaacgtgttccacacaatgtggcatgtcaccaggggagctgtactcatgtaccaagggaagagactggaaccgagctgggccagtgtcaaaaaagacctgatctcatatggaggaggttggaggcttcaaggatcctggaacacgggagaagaagtgcaggtgattgctgttgaaccagggaagaatcccaaaaatgtacaaacagcgccgggcacttttaagacccctgaaggtgaagttggagccattgccctagattttaaacccggcacatctggatctcccatcgtgaacagagaagggaaagtagtaggtctttatggaaatggagtggtgacaacaagtggaacctacgtcagtgccatagctcaagccaaagcatcacaagaagggcccctaccagagattgaagatgaggtgtttaggaaaagaaacttaacaataatggacctgcatccaggatcgggaaaaacaagaagatacctaccagctatagtccgtgaggccataaaaaggaagctgcgcacactaattctggctcccacaagggttgtcgcttccgaaatggcagaggcgctcaagggaatgccaataaggtaccaaacaacagcagtgaagagtgaacacacaggaaaagagatagttgacctcatgtgtcacgccaccttcaccatgcgcctcctgtctcccgtgagagttcccaattataacatgattattatggatgaagcacatttcaccgatccatccagcatagcggctagagggtacatctcaacccgagtgggcatgggtgaagcagctgcgattttcatgacagccactcccccaggatcagtggaggcctttccacagagcaacgcagttatccaagatgaggaaagagatattcctgagagatcatggaactcaggttatgagtggatcactgacttcccaggcaaaacagtttggtttgttccaagcattaaatcaggaaatgatattgccaactgcttaagaaagaatgggaaacgggtgattcaattgagcagaaaaacctttgacacagagtaccaaaaaacaaaaaataacgactgggactacgtcgtcacaacagacatctccgaaatgggagcaaatttccgggccgacagggtgatagacccaagacggtgtctgaaaccggtaatactaaaagatggtccagagcgtgtcatcttagcaggaccgatgccagtgactgtggctagtgccgcccagaggagaggaagaattggaaggaaccacaacaaggaaggtgatcagtacatctatatgggacagcctttaaacaacgatgaagatcacgctcactggacggaagcaaaaatgctccttgataatataaacacaccagaaggaattatcccagccctcttcgagccggagagagaaaagagtgcggcaatagatggggaatacagactgcggggtgaagcaaggaaaacgtttgtggagctcatgagaagaggagatctacctgtctggctatcctacaaagttgcctcagaaggcttccaatactctgacagaagatggtgctttgacggggaaaggaacaaccaggtgttggaagagaacatggacgtggagatctggacaaaagaaggagaaagaaagaaactacgaccccgctggctggatgccagaacatactcagacccactggccctgcgcgagtttaaagagtttgcagcaggaagaagaagcgtctcaggtgatctaatactggaaatagggaaacttccacaacacttgacgcaaagggcccagaatgccttggataacctggtcatgttgcacaactccgaacaaggaggaagagcctatagacatgcaatggaagaactgccagacaccatagaaacgttaatgctcctagctttgatagctgtgttaactggtggagtgacgctgttcttcctatcaggaaggggcttagggaaaacatctatcggcctactctgcgtgatggcttcaagcgtattgctatggatggccagtgtagagccccattggatagcggcctccatcatactggagttcttcctgatggtgctgctcattccagagccagacagacaacgcactccgcaggacaatcagctggcatatgtggtgataggtttgttattcatgatactaacagtagcagccaatgagatgggactgctggaaactacaaagaaagacttagggattggccatgtggctgttgaaaaccaccaccatgccacaatgctggacgtagacttacatccagcttcagcctggaccctctatgcagtggccacaacaatcatcactcccatgatgaggcacacaatcgaaaacacaacggcaaacatttccctgacagccgttgcaaatcaggcagctatattgatgggacttgacaaaggatggccaatatcgaagatggacataggagttccacttctcgccttggggtgttattcccaggtgaatccactgacgctgacagcggcggtattgatgctagtggcccattacgctataattggacctggactgcaagcaaaagctactagagaagctcaaaaaaggacagcggccggaataatgaaaaatccaactgttgatggaatcgttgcaatagacttggaccctgtggtttatgatgcgaaatttgagaaacaactaggccaaataatgttgttgatactatgcacatcacagatcctcttgatgcggactacatgggccttgtgcgaatccatcacactggccactggacctctgaccacgctctgggagggatctccaggaaaattttggaacaccacgatagcagtttccatggcaaacattttcagaggaagttatctagcaggagcaggtctggctttctcattaatgaaatctctaggaggaggtaggagaggcacgggagcccaaggggaaacactgggagagaaatggaaaagacagctgaaccaactgagcaagtcagaattcaacacctataaaaggagtgggattatggaagtggacagatccgaagccaaagagggactgaaaagaggagaaacaaccaaacatgcagtgtcgagaggaaccgctaaattgaggtggtttgtggagaggaaccttgtgaaaccagaagggaaagtcatagacctcggttgtggaagaggtggctggtcatactattgcgctgggctgaagaaagtcacagaggtgaagggatacacaaaaggaggacctggacacgaagaaccaatcccaatggcgacctatggatggaacctagtaaagctgtactccgggaaagacgtattttttataccacctgagaaatgtgacaccctcttgtgtgatattggtgagtcctctccaaacccaactatagaggaaggaagaacgctacgcgtcctaaagatggtggaaccatggctcagaggaaaccaattttgcataaaaattctgaatccctacatgccaagtgtggtggaaactctggagcaaatgcaaagaaaacatggaggaatgctggtgcgaaatccactttcaagaaattccactcatgaaatgtattgggtttcatgtggaacaggaaacattgtgtcagcagtaaacatgacatccagaatgttgctaaatcggttcacaatggctcataggaaaccaacatacgaaagagacgtggacctaggcgccggaacaagacatgtggcagtagaaccagaggtagctaacctagatatcattggccagaggatagagaacataaaacatgaacacaagtcaacatggcattatgatgaggacaatccatataaaacatgggcctatcatggatcatatgaggtcaaaccatcaggatcagcctcatccatggtcaatggtgtggtgaaactgctcaccaaaccatgggatgtcatccccatggtcacacaaatagctatgactgacactacaccctttggacaacagagggtatttaaagagaaagttgacacacgcacaccaaaagcaaaacgaggcacagcacaaatcatggaggtgacagccaggtggttatggggttttctttctagaaacaagaagccaagaatttgtacaagagaggagttcacaagaaaagttaggtcaaacgcagccatcggagcagtgttcattgacgaaaaccaatggaactcagcaaaagaagcagtggaagatgagcggttctgggaccttgtgcacagagagagggagcttcacaaacagggaaaatgtgctacgtgtgtttacaacatgatggggaagagagagaaaaagctaggagaatttggaaaggcaaaaggaagtcgtgcaatatggtacatgtggttgggagcacgctttctagagttcgaagctcttggtttcatgaacgaagaccactggttcagcagagagaattcactcagcggagtggaaggagaaggactccacaaacttggatatatactcagagacatatcaaagattccagggggaaacatgtacgctgatgacacagccggatgggatacaaggataacagaggacgaccttcagaatgaggccaaaattactgacatcatggaacccgaacatgccctactggctaaggcaatcttcaagctaacctaccaaaataaagtggtaagggtacagagaccagcaaaaaatggaaccgtgatggatgtcatatccagacgtgaccagagaggaagtggccaggtcggaacttatggcttaaacactttcaccaacatggaagcccagctgataagacaaatggagtctgagggaatcttttcacccagtgaattagagaccccaaatttagccgagagagttctcgactggttggaaaaatatggcgtcgaaaggctaaaaagaatggcaatcagtggagatgactgcgtagtgaaaccaattgatgataggtttgcaacagccttaacagctctgaatgatatgggaaaagtaagaaaagatataccacaatgggaaccctcaaaaggatggaatgattggcaacaagtgcctttttgttcacaccacttccaccagctgattatgaaggatgggagggaaatagtggtgccatgccgcaaccaagatgaacttgtgggtagggctagagtatcacaaggtgctggatggagcctgagagaaaccgcatgcctaggcaaatcatatgcacaaatgtggcagctgatgtacttccacaggagagacctgagactagctgctaatgctatctgttcagccgttccagttgattgggtcccaactagccgcaccacctggtctatccatgcccatcaccaatggatgacaacagaagacatgctgtcagtgtggaatagagtttggatagaggaaaacccatggatggaggacaaaacccatatatccagttgggaagatgttccatatttagggaaaagggaagatcaatggtgtggatccctgataggcttaacagcaagggccacctgggccaccaacatacaagtggccataaaccaagtgagaagactaattgggaatgagaattatctagattacatgacatcaatgaagagattcaagaacgagagtgatcccgaaggggcactttggtgagccaacacatttacaaaataaaggaaaataagaaatcaaacaaggcaagaagtcaggccggattaagccatagtacggtaagagctatgctgcctgtgagccccgtctaaggacgtaaaatgaagtcaggccgaaagccacggtttgagcaaaccgtgctgcctgtagctccatcgtggggatgtaaaaacctgggaggctgcaacccatggaagctgtacgcatggggtagcagactagtggttagaggagacccctcccgaaacacaacgcagcagcggggcccaacaccaggggaagctgtaccctggtggtaaggactagaggttagaggagaccccccgcataacaataaacagcatattgacgctgggagagaccagagatcctgctgtctctacagcatcattccaggcacagaacgccagaaaatggaatggtg

SEQ ID NO: 4 - DNA, 10594 bp, Artificial Sequence
  DENV2_ MF314189
tctacgtggaccgacaaagacagattctttgaggaagctaagcttaacgtagttctaacagttttttaattagagagcagatctctgatgaataaccaacggaaaaaggcgagaaatacgcctttcaatatgctgaaacgcgagagaaaccgcgtgtcaactgtgcagcagctgacaaagagattctcacttggaatgctacagggacgaggaccactgaaactgttcatggccctggtggcattccttcgtttcctaacaatcccgccaacagcagggatattaaaaagatggggaacaatcaaaaaatcaaaggctatcaatgtcttgagagggttcaggaaagagattggaaggatgctgaacatcttgaacaggagacgcagaactgcaggtataattattatgatgatcccaacagtgatggcgttccatttaaccacacgcaatggagaaccacacatgatcgtcagtagacaagagaaagggaaaagtcttctgtttaaaacagagaacggtgtgaacatgtgcaccctcatggccatggatcttggtgaactgtgtgaagacacaatcacttacaattgtcctcttctcaggcagaatgaaccagaagacatagactgttggtgcaactctacgtctacatgggtaacttatgggacatgcaccgctacaggagaacacagaagggaaaaaagatcagtggcactcgttccacatgtgggaatgggactggagacacgaactgaaacatggatgtcatcagaaggtgcctggaaacatgcacagagaattgaaacttgggtcttgagacatccaggcttcaccataatggcagcaatcctggcatacaccataggaacgacatatttccaaagagtcctgattttcatcttactgacagctgttgctccttcaatgacaatgcgttgtataggaatatcaaatagagactttgtggaaggggtttcaggaggaagctgggttgacatagtcctggaacatggaagctgtgtgacgacgatggcaaaaaataaaccaacattggattttgaactgataaagacagaagcgaaacatcccgccactctaaggaagtattgcatagaggcaaagctgaccaacacaacaacagcatctcgctgcccaacacaaggagaacctagcctaaatgaagaacaggacaaaagatttgtctgcaaacactccatggtagatagaggatggggaaatggatgcggattatttggaaagggaggtatcgtgacctgtgcaatgttcacatgcaaaaagaacatggaagggaaaatcgtgcaaccagaaaacttggagtacaccattgtgataacacctcactcaggggaagagaatgcagtcggaaatgacacaggaaaacacggcaaggaaattaaagtaacaccacagagttccatcacagaagcagaactaacaggctatggcactgtcacgatggaatgctctccgagaacgggactcgacttcaatgagatggtgttgctgcaaatggaaaacaaggcttggctggtgcacaggcaatggttcttagacctgccattaccatggctgcccggagcagacacacaaggatcaaattggatacagaaggagacattggtcactttcaaaaatccccatgcaaagaaacaggatgttgttgttctaggatcccaagaaggggctatgcacacagcacttacaggggccacggaaatccagatgtcatcaggaaacttactgttcacaggacatcttaaatgtaggctgagaatggacaaactacagctcaaaggaatgtcatattccatgtgtacaggaaagttcaaagttgtgaaggaaatagcagaaacacaacatggaacaatagttatcagagtacaatatgaaggggacggttctccgtgcaagatcccttttgaaataatggatttggaaaaaagacatgtcttaggtcgcttgatcacagtcaacccaattgtcacagaaaaagacagcccagtcaacatagaagcagaacctccattcggagacagctacatcattataggagtagaaccgggacaactgaagctcagctggtttaagaaaggaagctctattggccaaatgtttgagacaacaatgagaggagcgaagagaatggccattttaggtgacacagcttgggattttggatccctgggaggggtgttcacatctataggaaaggccctccaccaagtctttggagcaatctatggggctgccttcagtggggtttcatggactatgaaaatcctcataggagttgtcatcacatggataggaatgaattcacgtagcacttcactgtctgtgtcactagtattagtgggagtcgtgacattgtacttgggagttatggtgcaggccgatagtggttgcgttgtgagctggaaaaacaaagaactgaaatgtggcagcgggatttttatcacagacaacgtgcatacatggacagaacaatacaaattccaaccagaatccccttcaaagctggcttcagctatccagaaggctcatgaagaaggcatttgtggaatccgctcagtaacaagactggagaatctgatgtggaaacaaataacaccagaactgaatcacattttaacagaaaatgaggtaaagttgactatcatgacaggagacattaaaggaatcatgcaggcaggaaaacgatccctgcggcctcaacccactgagctgaagtactcttggaaagcatggggcaaagcgaaaatgctctccacagagcttcataaccacacctttctcattgatggccccgaaacagcagaatgtcccaacacaaatagagcttggaactcactagaggttgaagactatggctttggagtattcaccactaacatatggctgaaattgaaagaaaggcaggatgtatcttgtgactcaaaactcatgtcagcagccataaaagacaacagagccgtccacgccgacatgggttattggatagaaagcgcactcaatgacacatggaagattgagaaagcctcctttattgaagttaaaagctgccactggccaaagtcacacactctctggagtaatggagtgctagaaagtgagatgataattccaaagaattttgcaggaccagtgtcacaacacaattacagaccaggctatcatacacaaacggcaggaccctggcatctaggcaggcttgagatggactttgatttctgcgaaggaactacagtggtggtgactgaagactgtggaaatagaggaccctccttaagaacaactactgcttctggaaaactcataacagaatggtgctgccgatcttgcacattaccaccgctaaggtacagaggtgaggatggatgctggtatggaatggaaatcagaccattgaaagagaaagaagagaacttggtcaactctttggtcacagccggacatggacagattgacaacttctcactaggagtcttgggaatggcattgttcctggaagagatgcttagaacccgagtagggacgaaacatgcaatattactagttgcagtctctttcgtgacattgatcacagggaacatgtcctttcgagatttggggagagtgatggtcatggtgggcgctactatgacggatgacataggcatgggcgtgacctatcttgccctattagcagccttcaaggtcagaccaacttttgcagctggactactcttaagaaagctgacctccaaggaattgatgatgaccaccataggaatcgtactcctctctcagagcaccataccagaaaccatacttgaactgactgacgcgttggctttggggatgatggttctcaaaatagtaagaaacatggaaaagtatcaactagcagtgactatcatggctatcttgtgcgtcccaaatgcagtgatattacaaaacgcatggaaagtgagctgcacagcactggcagtggtgtccgtttccccactgcttttaacatcttcacagcagaaaacggattggataccactggcgttgacgatcaaaggccttaatccaacagccattttcttaacaaccctctcaagaactagcaagaaaaggagctggccactaaatgaggctattatggcagtcgggatggtgagcattttagccagttctttcttaaagaatgacattcccatgacaggaccactagtggctggagggcttctcactgtgtgttacgtgctcactggaagatcggctgatttggaactggagagagctgctgacataagatgggaagaacaggcagagatatcaggaagcagtccaattttgtcgataacaatatcggaagatggcagcatgtcgataaaaaatgaagaagaagaacaaacactgaccatactgattagaacaggactgctggtgatatcaggactttttcccgtgtcaataccaatcacggcagctgcatggtacctgtgggaagtgaaaaaacaacgagccggagtattgtgggatgtcccttcacctccacctgtgggaagggccgaactggaagatggagcctatagaatcaagcagaaagggattttgggatactcgcagataggagccggagtctacaaagaaggaactttccacacaatgtggcatgtcacacgtggtgctgttctaatgcataaagggaagagaattgaaccatcatgggcggacgtcaagaaggacctaatatcgtatggaggaggttggaagctagaaggagaatggaaggaaggagaagaagttcaggtcctggcattagagcctggaaagaatccaagagccgtccaaacaaaacccggtctttttaaaactaacactggaaccataggcgccgtatctctagacttttctcctggaacgtcaggatctccaattgtcgacaaaaaaggaaaagttgtgggcctttatggcaacggtgtcgtcacaaggagtggaacatacgtgagtgccatagcccagactgaaaaaagcattgaagacaacccagagattgaagatgacatctttcgaaagaaaagactgaccatcatggacctccacccaggagcaggaaaaacaaagagataccttccagcaatagtcagagaagccataaaacgaggcttgagaacactaatcctggcccccactagagttgtggcggctgaaatggaagaagctctcagaggacttccaataagatatcaaaccccagctatcaaagctgagcatactggacgggagattgtggatctaatgtgtcacgccacattcaccatgaggctactatcaccaattagagtgccaaattacaacctgattatcatggatgaagcccatttcacagacccagcaagcatagcggctagaggatacatctcaactcgagtagagatgggtgaagcagctgggattttcatgacagctacccctcctggaagcagagacccatttcctcagagcaacgcaccaatcatggatgaagaaagggaaattcctgagcgttcgtggaactctggacatgagtgggttacggattttaaagggaagactgtttggtttgttccaagtataaaagcaggaaatgatatagcagcttgcctgagaaagaatgggaagaaagtgatacaactcagcaggaagacctttgattctgaatatatcaagactaggaccaatgattgggactttgtggtcacgacagacatttcagaaatgggtgctaacttcaaggctgagagggttatagaccccagacgctgcatgaaaccagtcatactaacagacggtgaagagcgggttatcctggcaggacccatgccagtgacccactctagtgcagcacaaagaagagggagagtaggaagaaatccaaaaaatgaaaatgaccagtatatatacatgggggaacctctggaaaatgatgaagactgcgcacactggaaagaagctaagatgcttctagataacatcaacacgcctgaaggaatcattcccagcatgtttgaaccagagcgtgagaaggtcgacgccattgatggtgaataccgcttgagaggagaagcgaggaaaacatttgtggacctaatgagaagaggagacctaccagtttggctagcctacagagtggcagctgaaggtatcaactacgcagacagaagatggtgctttgatggagtcaggaacaaccaaatcttggaagaaaatgtggaagtggaaatttggacaaaagaaggagaaaggaagaaattaaaacccagatggttagatgctaggatctactctgacccactggcacttaaagaattcaaagaattcgcagctggaagaaaatccctgaccctgaatctaatcaccgagatgggtaggctcccaaccttcatgacccagaaagcaaggaatgcattggacaacttagcagtcctacacacggctgaagcaggcggaagagcgtacaatcatgctcttagtgaactgccggagactctggagacattgcttttactgacacttttagccacagtcacaggcggaatcttcctgttcttgatgagcggaaagggtatagggaagatgaccctgggaatgtgctgcatagtcacagctagcattcttctatggtatgcacaaatacagccacattggatagcagcttcaataatactggagttttttctcatagtcttgctcattccagaaccagaaaagcagagaacaccccaagataaccaattaacttatgttgtcatagccatccttacagtggtagccgcaaccatggcaaacgagatgggtttcctggaaaaaacaaagaaagatttcggattgggaagcatcacaacccagcaacctgagagcaacatcctggacatagatctacgtcctgcatcagcttggactctatatgctgtggcaacaactttcatcacaccaatgttgagacatagcattgaaaattcctcagtgaatgtgtctctaacagccattgccaaccaagccacagtgttaatgggtcttgggaaaggatggccattgtcgaaaatggacatcggagttccccttctcgctatcggatgctattcacaagttaaccccataaccctcacagcagcccttctcttattggtagcacattatgctatcatagggccaggactccaagcgaaagcaaccagagaggctcagaaaagagcagcagcgggcatcatgaaaaacccaactgtggatggaataacagtgattgacctagatccaataccatatgatccaaagtttgaaaagcagttgggacaagtaatgctcttagtcctctgcgtgactcaagtattgatgatgaggactacatgggctttatgtgaagctctaactttagcgaccgggcccatctctacactgtgggaaggaaatccagggagattttggaatacaactattgcagtgtcaatggctaacatttttagagggagttatctggccggagccggacttctcttttctatcatgaagaacacggccaacacaagaaggggaactggcaacacaggagaaacgcttggagagaaatggaaaaaccggttgaatgcattggggaagagtgaattccagatctataagaaaagtggaatccaggaagtggatagaacgttagcaaaagaaggcatcaggagaggagaaacggaccatcacgctgtgtcgcgaggctcagcgaaactgagatggttcgtcgagagaaaccttgtcacaccagaagggaaagtagtggaccttggctgcggcagggggggctggtcatactattgtgggggactaaagaatgtaaaggaagtcaaaggcctaacaaaaggaggaccaggacacgaagaacccattcccatgtcaacatatggttggaatctggtgcgtctgcaaagtggagtcgatgtcttttttactccgccagaaaagtgtgacacattgctgtgtgacataggggagtcgtcaccaaaccccacggttgaggcaggacgaacactcagagttctaaacttagtggaaaactggctgaacaataatacccaattttgcataaaggttcttaatccatatatgccttcagttatagaaaaaatggaagcgctacaaaggaaatacggaggagctttggtgaggaatccactctcacgaaattccacacacgagatgtactgggtatctaatgcttccgggaacatagtgtcatcagtgaacatgatttcaagaatgttgattaacagattcacaatgagacacaagaaggccacatacgagccggatgttgatctcggaagtggaacccgcaacatcggaattgaaagtgaagtaccaaacctagacataattgggaaaagaatagaaaaaataaaacaagagcatgaaacatcatggcactatgatcaagaccacccatacaaaacgtgggcctaccatggcagctacgaaacaaaacagactggatcagcatcatccatggtgaacggagtggttaggctgctaacaaaaccttgggacgtcatccccatggtgacacagatggcaatgacagacacgactccatttggacaacagcgcgttttcaaagagaaagtggacacgagaacccaagaaccaaaagaaggcacgaaaaaactaatgaaaatcacagcagaatggctctggaaagaactaggaaagaaaaagacacctaggatgtgcaccagagaagaatttacaagaaaggtgagaagcaatgcagccttaggtgccatattcactgatgagaacaagtggaagtcggcacgtgaagctgttgaagacagtggattttgggaattggttgacaaggaaaggaatctccatcttgaaggaaagtgtgagacatgtgtgtataacatgatgggaaagagagagaagaagctaggggagttcggcaaagcaaaaggcagcagagccatatggtacatgtggcttggagcacgcttcttagagtttgaagccctgggattcttgaatgaagatcactggttttccagagagaactccctgagtggagtagaaggagaagggctgcacaaactaggctacattctaagagacgtgagtaagaaagaaggaggagcaatgtacgccgatgacaccgcaggatgggacacaagaatcacgctagaggacttgaaaaatgaagaaatggtgacaaaccacatggaaggagaacacaagaaacttgctgaagccattttcagattaacgtaccaaaacaaagtggtgcgtgtgcaaagaccgacatcaagaggcacagtaatggacattatatcgagaagagaccaaagaggtagtggacaagttgtcacctacggcctcaatactttcaccaacatggaagcccaactgatcagacagatggagggagaaggagtcttcaaaagcatccagcacctgacagccacagaagaaattgcagtgaaaaactggttagtaagagtggggcgtgagaggttatcaagaatggccatcagcggagatgattgtgttgtgaaacccttagatgacaggtttgcaaacgctctaacagctttaaatgacatgggaaaggtcaggaaagacatacaacaatgggaaccttcaagaggatggaacgattggacacaagtgcccttttgttcacaccatttccatgagttaatcatgaaggacggtcgtgtacttgtggttccatgtagaaaccaagatgaactgattggtagggcccgaatttcccagggagccgggtggtccttgcgggaaacagcttgtttggggaagtcttacgcccaaatgtggagcctaatgtacttccacagacgtgaccttaggctggcggcaaacgccatttgctcggcagtcccttcacattgggttccaacaagtcgaacaacctggtccatacacgccacacatgagtggatgacaacagaagacatgctgacagtctggaacagggtgtggattcaagaaaacccatggatggaagacaaaactccagtagaatcatgggaggaaatcccatatttggggaagagagaagaccagtggtgcggctcattgattgggctaacaagcagggccacctgggcaaagaacatccaaacagcaataaatcaagttagatccctaataggcaatgaggaatacacagactacatgccatctatgaaaagattcagaagagaagaggaagaggcaggagtcttgtggtagaaagcaggaacatcgtgagacaaaatcagaagtcaggtcggattaagccatagtacggaaaaaactatgctacctgtgagccccgtccaaggacgttaaaagaagtcaggccactacaagtgccatagcttgagtaaactatgcagcctgtagctccacctgagaaggtgtaaaaaatctgggaggccacaaaccatggaagctgtacgcatggcgtagtggactagcggttagaggagacccctcctttacaaatcgcagcaacaatgggggcccaaggtgagatgaagctgtagtctcactgaaaggactagaggttagaggagacccc

SEQ ID NO: 5 - DNA, 10675 bp, Artificial Sequence
  DENV3_ KF954947
tttcgactcggaagcttgcttaacgtagtgctaacagtattttattagagagcagatctctgatgaacaaccaacggaagaagacgggaaaaccgtctatcaatatgctgaaacgcgtgagaaaccgtgtgtcaactggatcacagttggcgaagagattctcaaaaggattgctgaacggccagggaccaatgaaattggtcatggcgttcatagccttccttagatttctggccattccaccaacagcaggagttttggccagatggggaaccttcaagaagtcgggggccattaaggttctgaaaggcttcaagaaggagatttcaaacatgctgagcataatcaacaaacggaaaaagacatcgctctgtctcatgatgatattgccagcagcacttgctttccacttgacttcacgagatggagagccgcgcatgattgtggggaagaatgaaagaggaaaatccctactttttaagacagcctctggaatcaacatgtgcacactcatagccatggacttgggagaaatgtgtgatgacacggtcacttacaaatgcccccacattaccgaagtggaacctgaagacattgactgctggtgcaaccttacatcaacatgggtgacttatggaacgtgtaatcaagctggagagcatagacgcgacaagagatcagtggcgttagctccccatgtcggcatgggactggacacacgcacccaaacctggatgtcggctgaaggagcttggagacaagtcgagaaggtagagacatgggcccttaggcatccagggttcaccatactagccctatttcttgcccattacataggcacctccttgacccagaaggtggttatttttatactactaatgctggtcaccccatccatgacaatgagatgtgtgggagtgggaaacagagattttgtggaaggtctgtcaggagctacgtgggttgacgtggtgctagagcacggggggtgtgtgaccaccatggctaagaacaagcccacgctggatatagagcttcagaagaccgaggccacccaactggcgaccctaaggaagctatgcattgaggggaaaattaccaacataacaactgactcaagatgtcccacccaaggggaagcggttttgcctgaggagcaggaccagaactacgtgtgtaagcacacatacgtagatagaggctgggggaacggctgtggtttgttcggcaagggaagcttggtaacatgtgcgaaatttcaatgcctggaaccgatagagggaaaagtagtgcaatatgagaacctcaaatacaccgtcatcattacagtgcacacaggagaccaacaccaggtgggaaatgaaacgcagggaatcacggctgagataacgcctcaggcatcaactactgaagccatcttgcctgaatatggaacccttgggctagaatgctcaccacggacaggtttggacttcaatgaaatgatcttactaacaatgaagaacaaagcatggatggtacacagacaatggttttttgacctacctctaccatggacatcaggagccacaacagaaacaccaacttggaacaggaaggagctccttgtgacattcaaaaatgcacatgcgaaaaaacaagaagtagttgtccttggatcgcaagagggagcaatgcataccgcactgacaggagccacagaaatccaaaactcaggaggcacaagcatttttgcggggcacttaaagtgtagacttaagatggacaaattggaactcaaggggatgagctatgcaatgtgcacgaatacctttgtgttgaagaaagaagtctcagaaacgcagcatgggacaatactcattaaggtcgagtacaaaggggaagatgcaccttgcaagattcctttctccacagaggatggacaagggaaagctcacaatggcagactgatcacagccaacccagtggtgactaagaaggaggagcctgtcaacattgaggctgaacctccttttggggaaagtaatatagtaattggaattggagacaatgccttgaaaatcaattggtacaagaagggaagctctattgggaagatgttcgaggccactgccagaggtgcaaggcgcatggccatcttgggagacacagcttgggactttggatcagtgggtggtgttctgaactcattaggcaaaatggtgcaccaaatattcggaagtgcttacacagccctattcagtggagtctcttgggtgatgaaaattggaataggtgttctcttaacttggatagggttgaattcaaaaaacacatccatgtcattttcatgcattgcaataggaatcatcacactctatttgggagctgtggtacaagctgacatggggtgtgtcataaactggaaaggcaaagaacttaaatgcggaagtggaattttcgtcaccaacgaggtccatacctggacagagcagtacaaattccaagcggattccccaaaaagattggcgacagctattgtaggtgcttgggaaaatggagtgtgtggaattaggtcaacaaccagaatggagaatctcttgtggaagcaaatagccaatgaactgaactacatattatgggaaaacaacatcaaattaacggtagttgtgggcgacacaatcggggttttagagcaaggaaaaagaacactaacaccacaacccatggagctaaaatactcatggaaaacgtggggaaaggcaaaaatagtgacagctgaaacacaaaattcctctttcataatagacgggccaaacacaccggagtgtccaagtgcctcaagagcatggaatgtgtgggaggtggaagattacgggttcggagtcttcacaaccaacatatggctgaaactccgagaggtgtacacccaaatgtgtgaccataggctaatgtcggcagccgtcaaggatgagagggccgtgcatgccgacatgggctactggatagaaagccaaaagaatggaagttggaagctagaaaaagcatccctcatagaggtgaaaacctgcacatggccaaaatcacacactctttggagcaacggtgtgctagagagtgacatgatcattccaaagagtctagctggtcctatttcgcaacacaactacaggcccgggtaccacacccaaacggcaggaccctggcacttaggaaaattggagctggacttcaactattgtgaaggaacaacagttgtcatcacagaaaattgtgggacaagaggcccatcattgagaacgacaacagtgtcaggaaagttgatacatgaatggtgttgccgctcgtgcacacttcctcccctgcgatacatgggagaagacggctgttggtatggcatggaaatcagacccatcagtgagaaagaagagaacatggtaaagtctttagtctcagcgggaagtggaaaggtagacaacttcacaatgggtgtcttgtgtttggcaatcctctttgaagaggtgatgagaggaaaatttgggaagaaacacatgattgcaggggttttcttcacgtttgtgctccttctctcagggcaaataacatggagagacatggcgcacacactaataatgattgggtccaacgcctctgacaggatgggaatgggcgtcacctatctagctttaattgcaacatttaaaatccagccattcctggctttgggatttttcctaagaaaactgacatctagagaaaatttactgttaggagtcggactggctatggcaacaacgttacaattgccagaggacattgaacaaatggcaaatggaatcgccctggggctcatggctcttaaattgataacacaatttgaaacataccaattatggacagcattaatctccttaacgtgttcaaatacaattttcacgttgactgttgcttggagaacagccaccctgattttggccggagtttcacttttaccagtgtgccagtcttcgagcatgagaaaaacagactggcttccaatgacagtggcagctatgggagtcccacccctaccactctttatttttagcttgaaagacacactcaaaaggagaagctggccactgaatgagggggtgatggctgttggacttgtgagcatgctggccagttctctccttagaaatgacgtgcccatggctggaccattagtggccgggggcttgctgatagcgtgctacgtcataactggcacgtcagcagaccttacagtggaaaaagcagcagatgtaacatgggaggaagaggctgagcaaacaggagtgtcccacaacttaatgatcacagttgatgatgatggaacaatgagaataaaagatgatgagactgagaatattctaacagtgcttttgaagacagcattactaatagtatcaggtatctttccatactccataccagcgacattgttggtctggcatacttggcaaaagcaaacccaaagatccggtgttctatgggacgtacccagccccccagagacacagaaagcagaactggaagaaggggtctataggatcaaacagcaaggaattcttgggaaaacccaagtaggggttggagtacaaaaagacggagtcttccacaccatgtggcacgtcacaagaggggcagtgttgacacataatgggaaaagactggaaccaaactgggctagcgtgaaaaaagatctgatttcatacggaggaggatggagattgagcgcacaatggcaaaagggggaggaggtgcaggttattgccgtagagcctgggaagaatccaaagaacttccaaaccatgccaggcacattccagactacaacaggggaaataggagcaattgcattggatttcaagcctggaacttcagggtctcctatcataaacagagagggaaaggtagtgggactatatggcaatggagtggttacaaagaatggcggctacgtcagcggaatagcgcaaacaaatgcagaaccagatggaccgacgccagagttggaagaagagatgttcaaaaagcgaaatctaaccataatggatcttcatcctgggtcaggaaagacacggaaatatcttccagccattgttagagaggcaatcaagagacgtttaagaactctgattctggcaccgacaagggtggttgcagctgagatggaagaagcattgaaggggctcccaataaggtaccaaacaacagcaacaaaatctgaacatacgggaagagagattgttgatctaatgtgccacgcaacgttcacaatgcgcttgctgtcaccagttagggttccaaattacaacttgataataatggatgaggcccatttcacagacccagccagtatagcggccagagggtacatatcaactcgtgttggaatgggagaggcagccgcaatcttcatgacggcaacgccccctggaacagctgatgcctttcctcagagcaacgctccaattcaagatgaagaaagggacataccagaacgctcatggaattcaggcaatgaatggatcaccgacttcgccgggaaaacggtgtggtttgtccccagcatcaaagccggaaatgacatagcaaactgcttgcgaaagaacgggaaaaaggtcattcaacttagtaggaagacttttgatacagaatatcagaagactaaactaaatgactgggactttgtggtgacaactgacatttcagaaatgggggccaatttcaaagcagatagagtgatcgacccaagaagatgtctaaaaccagtgatcctgacagatggaccagagcgggtgatcctggctggaccaatgccagtcaccgcggcgagtgctgcgcaaaggagagggagagttggcaggaacccacaaaaagaaaatgaccagtacatattcacgggccagcctctcaacaatgacgaagaccatgctcactggacagaagcaaaaatgctgctggacaacatcaacactccagaaggaatcataccagctctctttgaaccagaaagggagaagtcagccgccatagacggtgaatatcgcctgaagggtgaatccaggaagactttcgtggaactcatgaggaggggtgacctcccagtttggttagcccacaaagtagcatcagaagggatcaaatatacagataggaaatggtgctttgatggacagcgcaacaatcaaattttagaggaaaacatggacgtggaaatctggacaaaggaaggagaaaagaaaaaattaagacctaggtggcttgatgcccgcacttattcagatcccttagcactcaaggaattcaaggactttgcggcaggcagaaagtcaatcgcccttgatcttgtgacagaaataggaagagtgccttcacacctagcccacagaacgagaaacgctctggacaatctggtgatgctgcacacgtcagaacatggcggtagggcctacaggcatgcggtggaggaactaccagaaacaatggaaacactcctactcttgggactcatgatcttactgacaggtggagcaatgcttttcttgatatcaggtaaagggattggaaagacttcaataggactcatttgtgtgattgcttccagcggcatgctgtggatggccgaaattccactccaatggatcgcgtcggctatagtcctggagttttttatgatggtgttgcttataccagaaccagaaaagcagagaaccccccaagacaaccaactcgcatatgtcgtaataggcatacttacaatggctgcaataatagcggccaatgaaatgggactattggaaactacaaagagagatctaggaatgtctaaggaaccaggtgttgtttctccaactagctatttggatgtggatttgcacccagcatcagcctggacattgtacgctgtggccactacagtaataacaccaatgttaagacataccatagagaattctacagcaaatgtgtccctggcagctatagccaaccaggcagtggtcctgatgggtttggacaaaggatggccaatatcaaaaatggacttaggcgtaccactactggcattgggttgctattcacaagtgaacccactgactctaacagcggcagtacttttgctagttacacattatgctattataggtccaggactgcaggcaaaagccactcgtgaagctcaaaaaaggacagctgctggaataatgaagaatccaacggtggatgggataataacaatagacctagaccctgtaatatatgattcaaaatttgaaaagcaactgggacaggtcatgctcctggttttgtgtgcagttcaactgttgttaatgagaacatcatgggccttgtgtgaagctttaactttagctacaggaccaataacaacactctgggaaggatcacctgggaagttttggaataccacgatagctgtttctatggcgaacatttttagagggagctatttagcaggagctgggcttgccttttctattatgaaatcagttggaacaggaaaaagaggaacaggctctcaaggtgaaactttaggagaaaaatggaaaaagaaattgaatcaattatcccggaaagagtttgacctttacaagaagtctggaatcactgaagtggatagaacagaagccaaagaagggttgaaaagaggagaaacaacacatcatgccgtgtccaggggtagtgcaaaacttcaatggtttgtggaaaggaacatggtcattcccgagggaagagtcatagacctgggctgtggaagaggaggctggtcatattactgtgcaggactgaaaaaagtcacagaagtgcgaggatacacaaaaggcggtccaggacacgaagaaccagtgcctatgtcaacatatggatggaacatagttaaattaatgagtggaaaggatgtgttttatcttccgcctgaaaagtgtgacaccctgttgtgtgacattggagaatcttcaccaagcccaacagtggaagaaagcagaactataagagttttgaagatggttgaaccatggctaaaaaacaaccagttttgcattaaagtattgaacccttacatgccagccgtgattgagcacctagaaagactgcaaaggaaacacggaggaatgcttgtgagaaatccactttcacgaaactccacgcacgaaatgtactggatatctaatggtacaggtaacattgtctcttcagttaacatggtatccagattgttactgaacaggttcacgatgacacacaggagacctaccatagagaaagatgtggatttaggagcaggaactcgacatgtcaatgcggaaccagaaacacccaacatggatgtcattggggaaagaataaaaaggatcaaggaggagcataattcaacatggcactatgatgacgaaaacccctacaaaacgtgggcttaccacggatcttatgaagtcaaggccacaggctcagcctcctccatgataaacggagtcgtgaaacttctcactaaaccatgggatgtagtgcccatggtgacacagatggcaatgacagatacaactccatttggccagcagagagtctttaaagagaaggtggacaccaggacacccaggcctatgccagggacaagaaaggttatggagatcacagcggagtggctctggagaaccctgggaaggaacaaaagacccaggttatgcacaagggaagagttcacaaaaaaggtcagaaccaacgcagccatgggcgccgttttcacagaggagaaccaatgggacagtgcgaaagccgctgttgaggatgaagagttttggaaacttgtggacagagaacgtgaactccacaaattgggcaagtgtggaagctgtgtttacaacatgatgggcaagagagagaagaaacttggagagtttggcaaagcaaaaggcagtagagctatatggtacatgtggttgggagccaggtaccttgagttcgaagcccttggattcttaaatgaagaccactggttctcgcgtgaaaactcttacagtggagtagaaggagaaggactgcacaagctaggctacatattaagggacatttccaagatacccggaggagccatgtatgctgatgacacagctggttgggacacaagaataacagaagatgacctgcacaatgaggaaaagatcacacaacgaatggaccctgaacacaggctgttagcgaacgctatatttaagctcacataccaaaacaaagtggtcaaagttcaacgaccgactccaacgggcacggtaatggacattatatctaggaaagaccaaagaggcagtggacaggtgggaacttatggtctgaacacatttactaacatggaagcccagttagtcagacaaatggaaggagaaggtgtgctgtcaaagacagacctcgagaaccctcatctgccagaaaagaaaattacacaatggctggaaaccaaaggagtggagaggttaaaaagaatggccattagcggggatgattgcgtagtgaaaccaatcgatgacaggttcgctaacgcactgcttgccctgaacgatatgggaaaggttcggaaagacatacctcaatggcagccatcaaagggatggcatgactggcagcaggttcctttctgctcccaccactttcatgaattgatcatgaaagatggaagaaagttggtggttccctgcagaccccaggacgaactaataggaagagcaagaatctctcaaggagcgggatggagccttagagaaaccgcatgtttggggaaagcctacgcccaaatgtggagtctcatgtattttcacagaagagatctcagactagcgtccaatgccatatgttcagcaataccagtccactgggtccccacaagtagaacgacatggtctattcatgctcaccatcagtggatgaccacagaagacatgcttactgtttggaacagggtgtggatcgaggacaatccatggatggaagacaaaactccaattacaacctgggaaaatgttccatacctagggaagagggaagaccaatggtgcggatcacttattggtctcacttccagagcaacctgggcccagaacatacccacagcaattcaacaggtgagaagccttataggcaatgaagagtttctggactacatgccttcaatgaagagattcaggaaggaggaggagtcggagggagccatttggtaaacgtaggaagtgaaaaagaggctgactgtcaggccaccttaagccacagtacggaagaagctgtgctgcctgtgagccccgtccaaggacgttaaaagaagaagtcaggccccaaagccacggtttgagcaaaccgtgctgcctgtagctccgtcgtggggacgtaaaacctgggaggctgcaaactgtggaagctgtacgcacagtgtagcagactagtggttagaggagacccctcccatgacacaacgcagcagcggggcccgagcactgagggaagctgtacctccttgcaaaggactagaggttagaggagaccccccgcaaacaaaaacagcatattgacgctgggagagaccagagatcctgctgtctcctcagcatcattccaggcacagaacgccagaaaatggaatggtgctgttgaatcaccaggttct

SEQ ID NO: 6 - DNA, 10649 bp, Artificial Sequence
  DENV4_ HQ332173
agttgttagtctgtgtggaccgacaaggacagttccaaatcggaagcttgcttaacacagttctaacagtttgtttgaatagagagcagatctctggaaaaatgaaccaacgaaaaaaggtggttagaccacctttcaatatgctgaaacgcgagagaaaccgcgtatcaacccctcaagggttggtgaagagattctcaaccggacttttttctgggaaaggacccttacggatggtgctagcattcatcacgtttttgcgagtcctttccatcccaccaacagcagggattctgaagagatggggacagttgaagaaaaataaggctatcaagatactgattggattcaggaaggagataggccgcatgctgaacatcttgaacgggagaaaaaggtcaacgataacattgttgtgcttgattcccaccgtaatggcgtttcacttgtcaacaagagatggcgaacccctcatgatagtggcaaaacatgaaagggggagacctctcttgtttaagacaacagaggggatcaacaaatgcactctcattgccatggacttgggtgaaatgtgtgaggacactgtcacgtataaatgccccctactggtcaataccgaacctgaagacattgattgctggtgcaacctcacgtctgcctgggtcatgtatgggacatgcacccagagcggagaacggagacgagagaagcgctcagtagctttaacaccacattcaggaatgggattggaaacaagagctgagacatggatgtcatcggaaggggcttggaagcatgctcagagagtagagagctggatactcagaaacccaggatttgcactcctggcaggatttatggcttatatgattgggcaaacagggatccagcgaactgtcttctttgtcctaatgatgctggtcgccccatcctacggaatgcgatgcgtaggagtaggaaacagagactttgtggaaggagtctcaggtggagcatgggtcgacctggtgctagaacatggaggatgcgtcacaaccatggcccagggaaaaccaaccttggattttgaactgaccaagacaacagccaaggaagtggctctgttaagaacctattgcattgaagccttaatatcaaacataactacggcaacaagatgtccaacgcaaggagagccttatctgaaagaggaacaggaccaacagtacatttgccggagagatgtggtagatagaggatggggcaatggctgtggcttgtttggaaaaggaggagttgtgacatgtgcgaagttctcatgttcggggaagataacaggcaatctggtccaaattgagaaccttgaatacacagtggttgtaacagtccacaatggagacacccatgcagtaggaaatgacacatccaatcatggagttacagccacgataactcccaggtcaccatcggtagaagtcaaactgccggactatggagaactaacactcgattgtgaacccaggtctggaattgacttcaatgagatgatcctaatgaaaatgaaaaagaaaacatggctcgtgcataagcaatggtttttggatctgcctcttccatggacaacaggagcagatacatcagaggttcactggaattacaaagagagaatggtgacatttaaggttcctcatgccaagagacaggatgtgacagtgctgggatctcaggaaggagccatgcattctgcccttgctggagccacagaagtggactccggtgatggaaatcacatgtttgcaggacatctcaagtgcaaagtccgtatggagaaattgagaatcaagggaatgtcatacacgatgtgttcaggaaagttttcaattgacaaagagatggcagaaacacagcatgggacaacagtggtgaaagtcaagtatgaaggtgctggagctccgtgtaaagtccccatagagataagagatgtaaacaaggaaaaagtggttgggcgcgttatctcagccacccctttggctgagaataccaacagtgtaaccaacatagaattagaacccccctttggggacagctacatagtgataggtgttggaaacagcgcactaacactccattggttcaggaaagggagttccattggcaagatgtttgagtccacatacagaggtgcaaaacgcatggccatcctaggtgaaacagcttgggattttggttccgttggtggactgttcacatcattgggaaaggctgtgcaccaggtttttggaagtgtgtatacaaccatgtttggaggagtctcatggatgattagaatcctaattgggttcttagtgttgtggattggcacgaactcaaggaacacttcaatggccatgacgtgcatagctgttggtggaatcactctgtttttgggcttcacggttcaagcggacatgggttgtgtggtgtcatggagtgggagagaattgaagtgtggaagcggaatttttgtggttgacaacgtgcacacttggacagaacagtacaaattccaaccagagtccccagcgagactagcgtctgcaatattaaatgcccacaaagacggggtctgtggaattagatcaaccacgaggctggaaaatgttatgtggaagcaaataaccaatgagctaaactatgttctctgggaaggaggacatgatctcactgtagtggctggggatgtgaaaggggtgttgaccaagggcaagagagcactcacacccccagcgagtgatctgaaatattcatggaagacatgggggaaagcaaaaatcttcacccctgaagcaagaaacagcacatttttaatagacggaccagacacctctgaatgccccaatgaacgaagagcatggaattcttttgaggtggaagactatggatttggcatgttcacgaccaacatatggatgaaattccgagaaggaagttcagaagtgtgtgaccacaggttaatgtcagctgcaattaaagaccagaaagctgtgcatgctgacatgggttattggatagagagctcaaaaaaccagacctggcagatagagagagcatctcttattgaagtgaaaacatgtctgtggcccaagacccatacactgtggagcaatggagtgctggaaagccagatgcttattccaaaatcatatgcgggccctttttcacagcacaattaccgccagggctatgctacgcaaaccgtgggtccatggcacttaggcaaactagagatagactttggagaatgccccggaacaacagtcacaattcaggagaattgtgaccatagaggcccatctttgaggaccaccactgcatctggaaaactagtcacgcaatggtgttgccgctcctgcacgatgccccccttaaggttcttaggagaagatgggtgctggtatgggatggagattaggcccttgagtgaaaaagaagagaacatggttaaatcacaggtgacggccggacagggcacatcggaaactttttctatgggtctgttgtgcctgaccttgtttgtggaagaatgcttgaggagaagagtcaccaggaaacacatgatattagctgtggtaatcactctttgtgctatcatcctggggggcctcacatggatggacttgctacgagccctcatcatgttgggggacactatgtctggtagaataggaggacagacccacctagccatcatggcagtgttcaagatgtcaccaggatacgtgctgggtgtgtttttaaggaaactcacttcaagagagacagcactaatggtaataggaatggccatgacaacaacactttcaattccacatgacctcatggaactcattgatggaatatcactaggactaattttgctaaaaatagtaacacagtttgacaacacccaagtgggaaccttagctctttccttgactttcataagatcaacaatgtcattggtcatggcttggaggaccattatggctgtgttgtttgtggtcacactcattcctttgtgcaggacaagctgtcttcaaaaacagtctcattgggtagaaataacagcactcatcctaggagcccaagctctgccagtgtacctaatgactcttatgaaaggagcctcaagaagatcttggcctcttaacgaaggcataatggctgtgggtttggttagtctcctaggaagcgctcttttaaagaatgatgtccctttggctggcccaatggtggcaggaggcttacttctggcggcttacgtaatgagtggcagctcagcagatctgtcactagagaaggccgctaatgtgcagtgggatgaaatggcagacataacaggctcaagtccaatcatagaagtgaagcaagatgaggatggctctttctccatacgggacgtcgaggaaaccaatatgataacccttttggtgaaactggcactgataacggtgtcaggtctctaccccttggcaattccaatcacaatgaccttatggtacatgtggcaagtgaaaacacaaagatcaggagccctgtgggacgtcccttcacccgctgccactcaaaaagccgcactgtctgaaggagtgtacaggatcatgcaaagagggttattcgggaaaactcaggttggagtagggatacacatggaaggtgtatttcacacaatgtggcatgttacaagaggatcggtgatctgccacgagactgggagattggagccatcttgggctgacgtcaggaatgatatgatatcatacggtgggggatggaggcttggagataaatgggacaaagaagaagacgttcaggtcctcgctatagaaccaggaaaaaatcccaaacatgtccaaacgaaacctggccttttcaagaccctgactggagaaattggagcagtaacattagatttcaaacccggaacgtctggttctcccattattaacaggaaaggaaaagtcatcggactctatggaaatggagtggttaccaaatcaggtgattacgtcagtgccataacgcaagccgaaaggattggagagccagattatgaagtggatgaggacattttccgaaagaaaagactaactataatggacttacaccccggagctggaaagacaaaaagaattcttccatcaatagtgagagaagccttaaaaaggaggctgcgaactttgattttggctcccacgagagtggtggcggccgagatggaagaggccctacgtggactgccaatccgttaccaaaccccagctgtaaaatcagaacacacaggaagagagattgtagacctcatgtgccatgcaaccttcacaacaagacttttgtcatcaaccagagttccaaactacaaccttatagtaatggatgaagcacatttcaccgatccttccagtgtcgcggctagaggatacatttcgaccagggtggaaatgggagaggcagcagccatcttcatgaccgcaacccctcccggagcgacagatccctttccccagagcaacagcccaatagaagacatcgagagagagattccggaaaggtcatggaacacagggttcgactggataacagactaccaagggaaaactgtgtggtttgttcccagcataaaagctggaaatgacattgcaaattgtttgagaaagtcgggaaagaaagttatccagttgagtaggaaaacctttgatacagaatatccaaaaacgaaactcacggactgggactttgtggtcactacagacatatctgaaatgggggctaactttagagctgggagagtgatagaccctagaagatgcctcaagccagttatcctaacagatgggccagagagagtcatcttagcaggtcctattccagtgactccagcaagcgctgctcagagaagagggcgaataggaaggaacccagcacaagaagacgaccaatacgttttctccggagacccactaaaaaatgatgaagatcatgcccactggacagaagcaaagatgctgcttgacaatatctacaccccagaagggatcattccaacattgtttggtccggaaagggaaaaaacccaagctattgatggagagtttcgcctcagaggggaacaaaggaagacttttgtggaattaatgaggagaggagaccttccggtgtggctgagttataaggtagcttctgctggcatttcttacaaagatcgggaatggtgcttcactggggaaagaaataaccaaattttagaagaaaacatggaggttgaaatttggactagagagggagaaaagaaaaaactgaggccaaaatggttagatgcacgtgtatacgctgaccctatggctttgaaggatttcaaggagtttgccagtggaaggaagagtataactctcgacatcctaacagagatcgccagtttgccaacttacctttcctctagggccaagctcgcccttgacaacatagtcatgctccacacaacagaaagaggagggagggcctatcaacacgccctgaacgaacttccggagtcactggaaacactcatgcttgtagccttactaggtgctatgacagcaggtatcttcctgtttttcatgcaagggaaaggaatagggaaattgtcaatgggtttgataaccattgcggtggctagtggcttgctctgggtagcagaaattcaaccccagtggatagcggcctcaatcatactggagttttttctcatggtactgttgataccagaaccagaaaaacaaaggaccccacaagacaatcaattgatctacgtcatattgaccattctcaccattattggtctaatagcagccaacgagatggggctgatagaaaaaacaaaaacggattttgggttttaccaggtaaaaacagaaaccaccatcctcgatgtggacctgagaccagcttcagcatggacgctctatgcggtagccaccacaattctgactcccatgctgagacacaccatagaaaatacgtcggccaacctatctttagcagccatcgccaaccaggcagccgtcctaatggggcttggaaaaggatggccactccacagaatggacctcggtgtgccgctgttagcaatgggatgctattctcaagtgaacccaacaaccttgacagcatccttagtcatgcttttagtccattatgcaataataggcccaggattgcaggcaaaagccacaagagaggcccagaaaaggacagctgctggaatcatgaaaaatcccacagtggacgggataacagtgatagatctagaaccaatatcctatgacccaaaatttgaaaagcaattagggcaggtcatgttactcgccttgtgtgctggacaactactcttgatgagaacaacatgggctttctgtgaagtcttgactttggccacaggaccaatcttgaccttgtgggagggcaacccgggaaggttttggaacacgaccatagccgtatctaccgccaacatttttaggggaagttacttggcaggagctggactggctttttcactcataaagaatgcacaaacccccaggaggggaactgggaccacaggagagacactgggagagaagtggaagagacagctaaactcattagacagaaaagagtttgaagagtataaaagaagtggaatactagaagtggacaggactgaagccaagtctgccctgaaagatgggtctaaaatcaagcatgcagtatctagagggtccagtaagatcagatggattgttgagagagggatggtaaagccaaaagggaaagttgtagatcttggctgtgggagaggaggatggtcttattacatggcgacactcaaaaacgtgactgaagtgaaagggtatacaaaaggaggtccaggacatgaagaaccgattcccatggctacttatggctggaatttggtcaaactccattcaggggttgacgtgttctacaaacccacagagcaagtggacaccctgctctgtgatattggggagtcatcttctaatccaacaatagaggaaggaagaacattaagagttttgaagatggtggagccatggctctcttcaaaacctgaattctgcatcaaagtccttaacccttacatgccaacagtcatagaagagctggagaaactgcagagaaaacatggtgggaaccttgtcagatgcccgctgtccaggaactccacccatgagatgtattgggtgtcaggagcgtcgggaaacattgtgagctctgtgaacacaacatcaaagatgttgttgaacaggttcacaacaaggcataggaaacccacttatgagaaggacgtagatcttggggcaggaacgagaagtgtctccactgaaacagaaaaaccagacatgacaatcattgggagaaggcttcagcgattgcaagaagagcacaaagaaacatggcattatgatcaggaaaacccatacagaacctgggcgtatcatgggagctatgaagctccttcgacaggctctgcgtcctccatggtgaacggggtggtgaaactgctaacaaaaccctgggatgtaattccaatggtgactcagttagccatgacagacacaaccccttttgggcaacaaagagtgttcaaagagaaggtggataccagaacaccgcaaccaaaaccaggcacacgaatggttatgaccacgacagccaattggctatgggccctccttggaaagaagaaaaatcccagactgtgcacaagggaagagttcatctcaaaagttaggtcaaacgcagccataggcgcagtctttcaagaggaacagggatggacatcagccagtgaagctgtgaatgacagccggttttgggaactggttgacaaagaaagggcccttcaccaagaagggaaatgtgaatcgtgtgtctataacatgatgggaaaacgtgagaaaaagttaggagagtttggcagagccaagggaagccgagcaatctggtatatgtggctgggagcgcggtttctggaatttgaagccctgggttttttgaatgaagatcactggtttggcagagaaaactcatggagtggagtggaaggggaaggtctgcacagattgggatacatcctggaggagatagacaagaaggatggagacctaatgtatgctgatgacacagcaggctgggacacaagaatcactgaggatgatcttcaaaatgaggaactgatcacggaacagatggctccccaccacaagatcctagccaaagccattttcaaactaacctatcaaaacaaagtggtgaaagtcctcagacccacaccgagaggagcggtgatggatatcatatccaggaaagaccagagaggtagtggacaagttggaacatatggtttgaacacattcaccaacatggaagttcaactcatccgccaaatggaagcagaaggagtcatcacacaagatgacatgcagaacccaaaagggttgaaagaaagagttgagaaatggctgagagagtgtggtgtcgacaggttaaagaggatggcaattagtggagacgattgcgtggtgaaacccctagatgagaggtttggcacttccctcctcttcttgaacgacatgggaaaggtgaggaaagatattccgcagtgggaaccatctaagggatggaaaaactggcaagaggttcctttttgctcccaccactttcacaagatctttatgaaggatggccgctcactagttgttccatgtagaaaccaggatgaactgatagggagagccagaatctcgcagggggctggatggagcttaagggaaacagcctgcctaggcaaagcttacgcccagatgtggtcgcttatgtacttccacagaagggatctgcgtctagcctccatggccatatgctcagcagttccaacggaatggtttccaacaagcagaacaacatggtcaatccatgctcaccaccaatggatgaccactgaagacatgctcaaggtgtggaacagagtgtggatagaagacaaccccaatatgattgacaagactccagtccattcgtgggaagatataccttacctagggaaaagagaggatttgtggtgtggatccctgattggactttcttctagagccacctgggcgaagaacattcacacggccataactcaggtcaggaatctgatcggaaaagaggaatacgtggactacatgccagtaatgaaaagatacagtgctccttcagagagtgaaggagttctgtaatcaccaacaacaaacaccaaaggctattgaagtcaggccacttgtgccacggtttgagcaaaccgtgctgcctgtagctccgccaataatgggaggcgtaataatccctagggaggccatgcgccacggaagctgtacgcgtggcatattggactagcggttagaggagacccctcccatcactgacaaaacgcagcaaaagggggcccgaagccaggaggaagctgtactcctggtggaaggactagaggttagaggagacccccccaacacaaaaacagcatattgacgctgggaaagaccagagatcctgctgtctctacaacatcaatccaggcacagagcgccgcaagatggattggtgttgttgatccaacaggttct

SEQ ID NO: 7 - DNA, 10272 bp, Artificial Sequence
  Zikavirus_ KU501216
atgaaaaacccaaaaaagaaatccggaggattccggattgtcaatatgctaaaacgcggagtagcccgtgtgagcccctttgggggcttgaagaggctgccagccggacttctgctgggtcatgggcccatcaggatggtcttggcgattctagcctttttgagattcacggcaatcaagccatcactgggtctcatcaatagatggggttcagtggggaaaaaagaggctatggaaataataaagaagttcaagaaagatctggctgccatgctgagaataatcaatgctaggaaggagaagaagagacgaggcgcagatactagtgtcggaattgttggcctcctgctgaccacagctatggcagcggaggtcactagacgtgggagtgcatactatatgtacttggacagaaacgatgctggggaggccatatcttttccaaccacattggggatgaataagtgttatatacagatcatggatcttggacacatgtgtgatgccaccatgagctatgaatgccctatgctggatgagggggtggaaccagatgacgtcgattgttggtgcaacacgacgtcaacttgggttgtgtacggaacctgccatcacaaaaaaggtgaagcacggagatctagaagagctgtgacgctcccctcccattccactaggaagctgcaaacgcggtcgcaaacctggttggaatcaagagaatacacaaagcacttgattagagtcgaaaattggatattcaggaaccctggcttcgcgttagcagcagctgccatcgcttggcttttgggaagctcaacgagccaaaaagtcatatacttggtcatgatactgctgattgccccggcatacagcatcaggtgcataggagtcagcaatagggactttgtggaaggtatgtcaggtgggacttgggttgatgttgtcttggaacatggaggttgtgtcaccgtaatggcacaggacaaaccgactgtcgacatagagctggttacaacaacagtcagcaacatggcggagataagatcctactgctatgaggcatcaatatcagacatggcttcggacagccgctgcccaacacaaggtgaagcctaccttgacaagcaatcagacactcaatatgtctgcaaaagaacgttagtggacagaggctggggaaatggatgtggactttttggcaaagggagcctggtgacatgcgctaagtttgcatgctccaagaaaatgaccgggaagagcatccagccagagaatctggagtaccggataatgctgtcagttcatggctcccagcacagtgggatgatcgttaatgacacaggacatgaaactgatgagaatagagcgaaggttgagataacgcccaattcaccaagagccgaagccaccctggggggttttggaagcctaggacttgattgtgaaccgaggacaggccttgacttttcagatttgtattacttgactatgaataacaagcactggttggttcacaaggagtggttccacgacattccattaccttggcacgctggggcagacaccggaactccacactggaacaacaaagaagcactggtggagttcaaggacgcacatgccaaaaggcaaactgtcgtggttctagggagtcaagaaggagcagttcacacggcccttgctggagctctggaggctgagatggatggtgcaaagggaaggctgtcctctggccacttgaaatgtcgcctgaaaatggataaacttagattgaagggcgtgtcatactccttgtgtaccgcagcgttcacattcaccaagatcccggctgaaacactgcacgggacagtcacagtggaggtacagtacgcagggacagatggaccttgcaaggttccagctcagatggcggtggacatgcaaactctgaccccagttgggaggttgataaccgctaaccccgtaatcactgaaagcactgagaactctaagatgatgctggaacttgatccaccatttggggactcttacattgtcataggagtcggggagaagaagatcacccaccactggcacaggagtggcagcaccattggaaaagcatttgaagccactgtgagaggtgccaagagaatggcagtcttgggagacacagcctgggactttggatcagttggaggcgctctcaactcattgggcaagggcatccatcaaatttttggagctgctttcaaatcattgtttggaggaatgtcctggttctcacaaattctcattggaacgttgctgatgtggttgggtctgaacacaaagaatggatctatttcccttatgtgcttggccttagggggagtgttgatcttcttatccacagccgtctctgctgatgtggggtgctcggtggacttctcaaagaaggagacgagatgcggtacaggggtgttcgtctataacgacgttgaagcctggagggacaggtacaagtaccatcctgactccccccgtagattggcagcagcagtcaagcaagcctgggaagatggtatctgcgggatctcctctgtttcaagaatggaaaacatcatgtggagatcagtagaaggggagctcaacgcaatcctggaagagaatggagttcaactgacggtcgttgtgggatctgtaaaaaaccccatgtggagagctccacagagattgcccgtgcctgtgaacgagctgccccacggctggaaggcttgggggaaatcgtacttcgtcagagcagcaaagacaaataacagctttgtcgtggatggtgacacactgaaggaatgcccactcaaacatagagcatggaacagctttcttgtggaggatcatgggttcggggtatttcacactagtgtctggctcaaggttagagaagattattcattagagtgtgatccagccgttattggaacagctgttaagggaaaggaggctgtacacagtgatctaggctactggattgagagtgagaagaatgacacatggaggctgaagagggcccatctgatcgagatgaaaacatgtgaatggccaaagtcccacacattgtggacagatggaatagaagagagtgatctgatcatacccaagtctttagctgggccactcagccatcacaataccagagagggctacaggacccaaatgaaagggccatggcacagtgaagagcttgaaattcggtttgaggaatgcccaggcactaaggtccacgtggaggaaacatgtggaacaagaggaccatctctgagatcaaccactgcaagcggaagggtgatcgaggaatggtgctgcagggagtgcacaatgcccccactgtcgttccgggctaaagatggctgttggtatggaatggagataaggcccaggaaagaaccagaaagcaacttagtaaggtcaatggtgactgcaggatcaactgatcacatggatcacttctcccttggagtgcttgtgattctgctcatggtgcaggaagggctaaagaagagaatgaccacaaagatcatcataagcacatcaatggcagtgctggtagctatgatcctgggaggattttcaatgagtgacctggctaagcttgcaattttgatgggtgccaccttcgcggaaatgaacactggaggagatgtagctcatctggcgctgatagcggcattcaaagtcagaccagcgttgctggtatctttcatcttcagagctaattggacaccccgtgaaagcatgctactggccttggcctcgtgtcttttgcaaactgcgatctccgccttggaaggcgacctgatggttctcatcaatggttttgctttggcctggttggcaatacgagcgatggttgttccacgcactgataacatcaccttggcaatcctggctgctctgacaccactggcccggggcacactgcttgtggcgtggagagcaggccttgctacttgcggggggtttatgctcctctctctgaagggaaaaggcagtgtgaagaagaacttaccatttgtcatggccctgggactaaccgctgtgaggctggtcgaccccatcaacgtggtgggactgctgttgctcacaaggagtgggaagcggagctggccccctagcgaagtactcacagctgttggcctgatatgcgcattggctggagggttcgccaaggcagatatagagatggctgggcccatggccgcggtcggtctgctaattgtcagttacgtggtctcaggaaagagtgtggacatgtacattgaaagagcaggtgacatcacatgggaaaaagatgcggaagtcactggaaacagtccccggctcgatgtggcgctagatgagagtggtgatttctccctggtggaggatgacggtccccccatgagagagatcatactcaaggtggtcctgatgaccatctgtggcatgaacccaatagccataccctttgcagctggagcgtggtacgtatacgtgaagactggaaaaaggagtggtgctctatgggatgtgcctgctcccaaggaagtaaaaaagggggagaccacagatggagtgtacagagtaatgactcgtagactgctaggttcaacacaagttggagtgggagttatgcaagagggggtctttcacactatgtggcacgtcacaaaaggatccgcactgagaagcggtgaagggagacttgatccatactggggagatgtcaagcaggatctggtgtcatactgtggtccatggaagctagatgccgcctgggacgggcacagcgaggtgcagctcttggccgtgccccccggagagagagcgaggaacatccagactctgcccggaatatttaagacaaaggatggggacattggagcggttgcgctggattacccagcaggaacttcaggatctccaatcctagacaagtgtgggagagtgataggactttatggcaatggggtcgtgatcaaaaatgggagttatgttagtgccatcacccaagggaggagggaggaagagactcctgttgagtgcttcgagccttcgatgctgaagaagaagcagctaactgtcttagacttacatcctggagctgggaaaaccaggagagttcttcctgaaatagtccgtgaagccataaaaacaagactccgtactgtgatcttagctccaaccagggttgtcgctgctgaaatggaggaggcccttagagggcttccagtgcgttatatgacaacagcagtcaatgtcacccactctggaacagaaatcgtcgacttaatgtgccatgccaccttcacttcacgtctactacagccaatcagagtccccaactataatctgtatattatggatgaggcccacttcacagatccctcaagtatagcagcaagaggatacatttcaacaagggttgagatgggcgaggcggctgccatcttcatgaccgccacgccaccaggaacccgtgacgcatttccggactccaactcaccaattatggacaccgaagtggaagtcccagagagagcctggagctcaggctttgattgggtgacggatcattctggaaaaacagtttggtttgttccaagcgtgaggaacggcaatgagatcgcagcttgtctgacaaaggctggaaaacgggtcatacagctcagcagaaagacttttgagacagagttccagaaaacaaaacatcaagagtgggactttgtcgtgacaactgacatttcagagatgggcgccaactttaaagctgaccgtgtcatagattccaggagatgcctaaagccggtcatacttgatggcgagagagtcattctggctggacccatgcctgtcacacatgccagcgctgcccagaggagggggcgcataggcaggaatcccaacaaacctggagatgagtatctgtatggaggtgggtgcgcagagactgacgaagaccatgcacactggcttgaagcaagaatgctccttgacaatatttacctccaagatggcctcatagcctcgctctatcgacctgaggccgacaaagtagcagccattgagggagagttcaagcttaggacggagcaaaggaagacctttgtggaactcatgaaaagaggagatcttcctgtttggctggcctatcaggttgcatctgccggaataacctacacagatagaagatggtgctttgatggcacgaccaacaacaccatactggaagacagtgtgccggcagaggtgtggaccagacacggagagaaaagagtgctcaaaccgaggtggatggacgccagagtttgttcagatcatgcggccctgaagtcattcaaggagtttgccgctgggaaaagaggagcggcttttggagtgatggaagccttgggaacactgccaggacacatgacagagagattccaggaagccattgacaacctcgctgtgctcatgcgggcagagactggaagcaggccttacaaagccgcggcggcccaattgccggagaccctagagaccattatgcttttggggttgctgggaacagtctcgctgggaatctttttcgtcttgatgaggaacaagggcatagggaagatgggctttggaatggtgacccttggggccagtgcatggctcatgtggctctcggaaattgagccagccagaattgcatgtgtcctcattgttgtgttcctattgctggtggtgctcatacctgagccagaaaagcaaagatctccccaggacaaccaaatggcaatcatcatcatggtagcagtaggtcttctgggcttgattaccgccaatgaactcggatggttggagagaacaaagagtgacctaagccatctaatgggaaggagagaggagggagcaaccataggattctcaatggacattgacctgcggccagcctcagcttgggccatctatgctgccttgacaactttcattaccccagccgtccaacatgcagtgaccacttcatacaacaactactccttaatggcgatggccacgcaagctggagtgttgtttggtatgggcaaagggatgccattctacgcatgggactttggagtcccgctgctaatgataggttgctactcacaattaacacccctgaccctaatagtggccatcattttgctcgtggcgcactacatgtacttgatcccagggctgcaggcagcagctgcgcgtgctgcccagaagagaacggcagctggcatcatgaagaaccctgttgtggatggaatagtggtgactgacattgacacaatgacaattgacccccaagtggagaaaaagatgggacaggtgctactcatagcagtagccgtctccagcgccatactgtcgcggaccgcctgggggtggggggaggctggggccctgatcacagccgcaacttccactttgtgggaaggctctccgaacaagtactggaactcctctacagccacttcactgtgtaacatttttaggggaagttatttggctggagcttctctaatctacacagtaacaagaaacgctggcttggtcaagagacgtgggggtggaacaggagagaccctgggagagaaatggaaggcccgcttgaaccagatgtcggccctggagttctactcctacaaaaagtcaggcatcactgaggtgtgcagagaagaggcccgccgcgccctcaaggacggtgtggcaacgggaggccatgctgtgtcccgaggaagtgcaaagctgagatggttggtggagcggggatacctgcagccctatggaaaggtcattgatcttggatgtggcagagggggctggagttactacgccgccaccatccgcaaagttcaagaagtgaaaggatacacaaaaggaggccctggtcatgaagaacccgtgttggtgcaaagctatgggtggaacatagtccgtcttaagagtggggtggacgtctttcatatggcggctgagccgtgtgacacgttgctgtgtgacataggcgagtcatcatctagtcctgaagtggaagaagcacggacgctcagagtcctctccatggtgggggattggcttgaaagaagaccaggagccttttgtataaaagtgttgtgcccatacaccagcactatgatggaaaccctggagcgactgcagcgtaggtatgggggaggactggtcagagtgccactctcccgcaactctacacatgagatgtactgggtctctggagcgaaaagcaacaccataaaaagtgtgtccaccacgagccagctcctcttggggcgcatggacgggcctaggaggccagtgaaatatgaggaggatgtgaatctcggctctggcacgcgggctgtggtaagctgcgctgaagctcccaacatgaagatcattggtaaccgcattgaaaggatccgcagtgagcacgcggaaacgtggttctttgacgagaaccacccatataggacatgggcttaccatggaagctatgaggcccccacacaagggtcagcgtcctctctaataaacggggttgtcaggctcctgtcaaaaccctgggatgtggtgactggagtcacaggaatagccatgaccgacaccacaccgtatggtcagcaaagagttttcaaggaaaaagtggacactagggtgccagacccccaagaaggcactcgtcaggttatgagcatggtctcttcctggttgtggaaagagctaggcaaacacaaacggccacgagtctgtaccaaagaagagttcatcaacaaggttcgtagcaatgcagcattaggggcaatatttgaagaggaaaaagagtggaagactgcagtggaagctgtgaacgatccaaggttctgggctctagtggacaaggaaagagagcaccacctgagaggagagtgccagagttgtgtgtacaacatgatgggaaaaagagaaaagaaacaaggggaatttggaaaggccaagggcagccgcgccatctggtatatgtggctaggggctagatttctagagttcgaagcccttggattcttgaacgaggatcactggatggggagagagaactcaggaggtggtgttgaagggctgggattacaaagactcggatatgtcctagaagagatgagttgcataccaggaggaaggatgtatgcagatgacactgctggctgggacacccgcatcagcaggtttgatctggagaatgaagctctaatcaccaaccaaatggagaaagggcacagggccttggcattggccataatcaagtacacataccaaaacaaagtggtaaaggtccttagaccagctgaaaaagggaaaacagttatggacattatttcaagacaagaccaaagggggagcggacaagttgtcacttacgctcttaacacatttaccaacctagtggtgcaactcattcggaatatggaggctgaggaagttctagagatgcaagacttgtggctgctgcggaggtcagagaaagtgaccaactggttgcagagcaacggatgggataggctcaaacgaatggcagtcagtggagatgattgcgttgtgaagccaattgatgataggtttgcacatgccctcaggttcttgaatgatatgggaaaagttaggaaggacacacaagagtggaaaccctcaactggatgggacaactgggaagaagttccgttttgctcccaccacttcaacaagctccatctcaaggacgggaggtccattgtggttccctgccgccaccaagatgaactgattggccgggcccgcgtctctccaggggcgggatggagcatccgggagactgcttgcctagcaaaatcatatgcgcaaatgtggcagctcctttatttccacagaagggacctccgactgatggccaatgccatttgttcatctgtgccagttgactgggttccaactgggagaactacctggtcaatccatggaaagggagaatggatgaccactgaagacatgcttgtggtgtggaacagagtgtggattgaggagaacgaccacatggaagacaagaccccagttacgaaatggacagacattccctatttgggaaaaagggaagacttgtggtgtggatctctcatagggcacagaccgcgcaccacctgggctgagaacattaaaaacacagtcaacatggtgcgcaggatcataggtgatgaagaaaagtacatggactacctatccacccaagttcgctacttgggtgaagaagggtctacacctggagtgctgtaa

SEQ ID NO: 8 - DNA, 10862 bp, Artificial Sequence
  Yellowfevervirus_ JN628281
agtaaatcctgtgtgctaattgaggtgcattggtctgcaaatcgagttgctaggcaataaacacatttggattaattttaatcgttcgttgagcgattagcagagaactgaccagaacatgtctggtcgtaaagctcagggaaaaaccctgggcgtcaatatggtacgacgaggagttcgctccttgtcaaacaaaataaaacaaaaaacaaaacaaattggaaacagacctggaccttcaagaggtgttcaaggatttatctttttctttttgttcaacattttgactggaaaaaagatcacagcccacctaaagaggttgtggaaaatgctggacccaagacaaggcttggctgttctaaggaaagtcaagagagtggtggccagtttgatgagaggattgtcctcaaggaaacgccgttcccatgatgttctgactgtgcaattcctaattttgggaatgctgttgatgacgggtggagtgaccttggtgcggaaaaacagatggttgctcctaaatgtgacatctgaggacctcgggaaaacattctctgtgggcacaggcaactgcacaacaaacattttggaagccaagtactggtgcccagactcaatggaatacaactgtcccaatctcagtccaagagaggagccagatgacattgattgctggtgctatggggtggaaaacgttagagtcgcatatggtaagtgtgactcagcaggcaggtctaggaggtcaagaagggccattgacttgcctacgcatgaaaaccatggtttgaagacccggcaagaaaaatggatgactggaagaatgggtgaaaggcaactccaaaagattgagagatggttcgtgaggaaccccttttttgcagtgacggctctgaccattgcctaccttgtgggaagcaacatgacgcaacgagtcgtgattgccctactggtcttggctgttggtccggcctactcagctcactgcattggaattactgacagggatttcattgagggggtgcatggaggaacttgggtttcagctaccctggagcaagacaagtgtgtcactgttatggcccctgacaagccttcattggacatctcactagagacagtagccattgatagacctgctgaggtgaggaaagtgtgttacaatgcagttctcactcatgtgaagattaatgacaagtgccccagcactggagaggcccacctagctgaagagaacgaaggggacaatgcgtgcaagcgcacttattctgatagaggctggggcaatggctgtggcctatttgggaaagggagcattgtggcatgcgccaaattcacttgtgccaaatccatgagtttgtttgaggttgatcagaccaaaattcagtatgtcatcagagcacaattgcatgtaggggccaagcaggaaaattggactaccgacattaagactctcaagtttgatgccctgtcaggctcccaggaagtcgagttcattgggtatggaaaagctacactggaatgccaggtgcaaactgcggtggactttggtaacagttacatcgctgagatggaaacagagagctggatagtggacagacagtgggcccaggacttgaccctgccatggcagagtggaagtggcggggtgtggagagagatgcatcatcttgtcgaatttgaacctccgcatgccgccactatcagagtactggccctgggaaaccaggaaggctccttgaaaacagctcttactggcgcaatgagggttacaaaggacacaaatgacaacaacctttacaaactacatggtggacatgtttcttgcagagtgaaattgtcagctttgacactcaaggggacatcctacaaaatatgcactgacaaaatgttttttgtcaagaacccaactgacactggccatggcactgttgtgatgcaggtgaaagtgtcaaaaggagccccctgcaggattccagtgatagtagctgatgatcttacagcggcaatcaataaaggcattttggttacagttaaccccatcgcctcaaccaatgatgatgaagtgctgattgaggtgaacccaccttttggagacagctacattatcgttgggagaggagattcacgtctcacttaccagtggcacaaagagggaagctcaataggaaagttgttcactcagaccatgaaaggcgtggaacgcctggccgtcatgggagacaccgcctgggatttcagctccgctggagggttcttcacttcggttgggaaaggaattcatacggtgtttggctctgcctttcaggggctatttggcggcttgaactggataacaaaggtcatcatgggggcggtacttatatgggttggcatcaacacaagaaacatgacaatgtccatgagcatgatcttggtaggagtgatcatgatgtttttgtctctaggagttggggcggatcaaggatgcgccatcaactttggcaagagagagctcaagtgcggagatggtatcttcatatttagagactctgatgactggctgaacaagtactcatactatccagaagatcctgtgaagcttgcatcaatagtgaaagcctcttttgaagaagggaagtgtggcctaaattcagttgactcccttgagcatgagatgtggagaagcagggcagatgagatcaatgccatttttgaggaaaacgaggtggacatttctgttgtcgtgcaggatccaaagaatgtttaccagagaggaactcatccattttccagaattcgggatggtctgcagtatggttggaagacttggggtaagaaccttgtgttctccccagggaggaagaatggaagcttcatcatagatggaaagtccaggaaagaatgcccgttttcaaaccgggtctggaattctttccagatagaggagtttgggacgggagtgttcaccacacgcgtgtacatggacgcagtctttgaatacaccatagactgcgatggatctatcttgggtgcagcggtgaacggaaaaaagagtgcccatggctctccaacattttggatgggaagtcatgaagtaaatgggacatggatgatccacaccttggaggcattagattacaaggagtgtgagtggccactgacacatacgattggaacatcagttgaagagagtgaaatgttcatgccgagatcaatcggaggcccagttagctctcacaatcatatccctggatacaaggttcagacgaacggaccttggatgcaggtaccactagaagtgaagagagaagcttgcccagggactagcgtgatcattgatggcaactgtgatggacggggaaaatcaaccagatccaccacggatagcgggaaagttattcctgaatggtgttgccgctcctgcacaatgccgcctgtgagcttccatggtagtgatgggtgttggtatcccatggaaattaggccaaggaaaacgcatgaaagccatctggtgcgctcctgggttacagctggagaaatacatgctgtcccttttggtttggtgagcatgatgatagcaatggaagtggtcctaaggaaaagacagggaccaaagcaaatgttggttggaggagtagtgctcttgggagcaatgctggtcgggcaagtaactctccttgatttgctgaaactcacagtggctgtgggattgcatttccatgagatgaacaatggaggagacgccatgtatatggcgttgattgctgccttttcaatcagaccagggctgctcatcggctttgggctcaggaccctatggagccctcgggaacgccttgtgctgaccctaggagcagccatggtggagattgccttgggtggcgtgatgggcggcctgtggaagtatctaaatgcagtttctctctgcatcctgacaataaatgctgttgcttctaggaaagcatcaaataccatcttgcccctcatggctctgttgacacctgtcactatggctgaggtgagacttgccgcaatgttcttttgtgccgtggttatcataggggtccttcaccagaatttcaaggacacctccatgcagaagactatacctctggtggccctcacactcacatcttacctgggcttgacacaaccttttttgggcctgtgtgcatttctggcaacccgcatatttgggcgaaggagtatcccagtgaatgaggcactcgcagcagctggtctagtgggagtgctggcaggactggcttttcaggagatggagaacttccttggtccgattgcagttggaggactcctgatgatgctggttagcgtggctgggagggtggatgggctagagctcaagaagcttggtgaagtttcatgggaagaggaggcggagatcagcgggagttccgcccgctatgatgtggcactcagtgaacaaggggagttcaagctgctttctgaagagaaagtgccatgggaccaggttgtgatgacctcgctggccttggttggggctgccctccatccatttgctcttctgctggtccttgctgggtggctgtttcatgtcaggggagctaggagaagtggggatgtcttgtgggatattcccactcctaagatcatcgaggaatgtgaacatctggaggatgggatttatggcatattccagtcaaccttcttgggggcctcccagcgaggagtgggagtggcacagggaggggtgttccacacaatgtggcatgtcacaagaggagctttccttgtcaggaatggcaagaagttgattccatcttgggcttcagtaaaggaagaccttgtcgcctatggtggctcatggaagttggaaggcagatgggatggagaggaagaggtccagttgatcgcggctgttccaggaaagaacgtggtcaacgtccagacaaaaccgagcttgttcaaagtgaggaatgggggagaaatcggggctgtcgctcttgactatccgagtggcacttcaggatctcctattgttaacaggaacggagaggtgattgggctgtacggcaatggcatccttgtcggtgacaactccttcgtgtccgccatatcccagactgaggtgaaggaagaaggaaaggaggagctccaagagatcccgacaatgctaaagaaaggaatgacaactgtccttgattttcatcctggagctgggaagacaagacgtttcctcccacagatcttggccgagtgcgcacggagacgcttgcgcactcttgtgttggcccccaccagggttgttctttctgaaatgaaggaggcttttcacggcctggacgtgaaattccacacacaggctttttccgctcacggcagcgggagagaagtcattgatgctatgtgccatgccaccctaacttacaggatgttggaaccaactagggttgttaactgggaagtgatcattatggatgaagcccattttttggatccagctagcatagccgctagaggttgggcagcgcacagagctagggcaaatgaaagtgcaacaatcttgatgacagccacaccgcctgggactagtgatgaatttccacattcaaatggtgaaatagaagatgttcaaacggacatacccagtgagccctggaacacagggcatgactggatcctggctgacaaaaggcccacggcatggttccttccatccatcagagctgcaaatgtcatggctgcctctttgcgtaaggctggaaagagtgtggtggtcctgaacaggaaaacctttgagagagaataccccacgataaagcagaagaaacctgactttatattggccactgacatagctgaaatgggagccaacctttgcgtggagcgagtgctggattgcaggacggcttttaagcctgtgcttgtggatgaagggaggaaggtggcaataaaagggccacttcgtatctccgcatcctctgctgctcaaaggagggggcgcattgggagaaatcccaacagagatggagactcatactactattctgagcctacaagtgaaaataatgcccaccacgtctgctggttggaggcctcaatgctcttggacaacatggaggtgaggggtggaatggtcgccccactctatggcgttgaaggaactaaaacaccagtttcccctggtgaaatgagactgagggatgaccagaggaaagtcttcagagaactagtgaggaattgtgacctgcccgtttggctttcgtggcaagtggccaaggctggtttgaagacgaatgatcgtaagtggtgttttgaaggccctgaggaacatgagatcttgaatgacagcggtgaaacagtgaagtgcagggctcctggaggagcaaagaagcctctgcgcccaaggtggtgtgatgaaagggtgtcatctgaccagagtgcgctgtctgaatttattaagtttgctgaaggtaggaggggagctgctgaagtgctagttgtgctgagtgaactccctgatttcctggctaaaaaaggtggagaggcaatggataccatcagtgtgtttctccactctgaggaaggctctagggcttaccgcaatgcactatcaatgatgcctgaggcaatgacaatagtcatgctgtttatactggctggactactgacatcgggaatggtcatctttttcatgtctcccaaaggcatcagtagaatgtctatggcgatgggcacaatggccggctgtggatatctcatgttccttggaggcgtcaaacccactcacatctcctatatcatgctcatattctttgtcctgatggtggttgtgatccccgagccagggcaacaaaggtccatccaagacaaccaagtggcatacctcattattggcatcctgacgctggtttcagcggtggcagccaacgagctaggcatgctggagaaaaccaaagaggacctctttgggaagaagaacttaattccatctagtgcttcaccctggagttggccggatcttgacctgaagccaggagctgcctggacagtgtacgttggcattgttacaatgctctctccaatgttgcaccactggatcaaagtcgaatatggcaacctgtctctgtctggaatagcccagtcagcctcagtcctttctttcatggacaaggggataccattcatgaagatgaatatctcggtcataatgctgctggtcagtggctggaattcaataacagtgatgcctctgctctgtggcatagggtgcgccatgctccactggtctctcattttacctggaatcaaagcgcagcagtcaaagcttgcacagagaagggtgttccatggcgttgccaagaaccctgtggttgatgggaatccaacagttgacattgaggaagctcctgaaatgcctgccctttatgagaagaaactggctctatatctccttcttgctctcagcctagcttctgttgccatgtgcagaacgcccttttcattggctgaaggcattgtcctagcatcagctgccctagggccgctcatagagggaaacaccagccttctttggaatggacccatggctgtctccatgacaggagtcatgagggggaatcactatgcttttgtgggagtcatgtacaatctatggaagatgaaaactggacgccgggggagcgcgaatggaaaaactttgggtgaagtctggaagagggaactgaatctgttggacaagcgacagtttgagttgtataaaaggaccgacattgtggaggtggatcgtgatacggcacgcaggcatttggccgaagggaaggtggacaccggggtggcggtctccagggggaccgcaaagttaaggtggttccatgagcgtggctatgtcaagctggaaggtagggtgattgacctggggtgtggccgcggaggctggtgttactacgctgctgcgcaaaaggaagtgagtggggtcaaaggatttactcttggaagagacggccatgagaaacccatgaatgtgcaaagtctgggatggaacatcatcaccttcaaggacaaaactgatatccaccgcctagaaccagtgaaatgtgacacccttttgtgtgacattggagagtcatcatcgtcatcggtcacagagggggaaaggaccgtgagagttcttgatactgtagaaaaatggctggcttgtggggttgacaacttctgtgtgaaggtgttagctccatacatgccagatgttctcgagaaactggaattgctccaaaggaggtttggcggaacagtgatcaggaaccctctctccaggaattccactcatgaaatgtactacgtgtctggagcccgcagcaatgtcacatttactgtgaaccaaacatcccgcctcctgatgaggagaatgaggcgtccaactggaaaagtgaccctggaggctgacgtcatcctcccaattgggacacgcagtgttgagacagacaagggacccctggacaaagaggccatagaagaaagggttgagaggataaaatctgagtacatgacctcttggttttatgacaatgacaacccctacaggacctggcactactgtggctcctatgtcacaaaaacctcaggaagtgcggcgagcatggtaaatggtgttattaaaattctgacatatccatgggacaggatagaggaggtcacaagaatggcaatgactgacacaaccccttttggacagcaaagagtgtttaaagaaaaagttgacaccagagcaaaggatccaccagcgggaactaggaagatcatgaaagttgtcaacaggtggctgttccgccacctggccagagaaaagaaccccagactgtgcacaaaggaagaatttattgcaaaagtccgaagtcatgcagccattggagcttacctggaagaacaagaacagtggaagactgccaatgaggctgtccaagacccaaagttctgggaactggtggatgaagaaaggaagctgcaccaacaaggcaggtgtcggacttgtgtgtacaacatgatggggaaaagagagaagaagctgtcagagtttgggaaagcaaagggaagccgtgccatatggtatatgtggctgggagcgcggtatcttgagtttgaggccctgggattcctgaatgaggaccattgggcttccagggaaaactcaggaggaggagtggaaggcattggcttacaatacctaggatatgtgatcagagacctggctgcaatggatggtggtggattctacgcggatgacaccgctggatgggacacgcgcatcacagaggcagaccttgatgatgaacaggagatcttgaactacatgagcccacatcacaaaaaactggcacaagcagtgatggaaatgacatacaagaacaaagtggtgaaagtgttgagaccagccccaggagggaaagcctacatggatgtcataagtcgacgagaccagagaggatccgggcaggtagtgacttatgctctgaacaccatcaccaacttgaaagtccaattgatcagaatggcagaagcagagatggtgatacatcaccaacatgttcaagattgtgatgaatcagttctgaccaggctggaggcatggctcactgagcacggatgtaacagactgaagaggatggcggtgagtggagacgactgtgtggtccggcccatcgatgacaggttcggcctggccctgtcccatctcaacgccatgtccaaggttagaaaggacatatctgaatggcagccatcaaaagggtggaatgattgggagaatgtgcccttctgttcccaccacttccatgaactacagctgaaggatggcaggaggattgtggtgccttgccgagaacaggacgagctcattgggagaggaagggtgtctccaggaaacggctggatgatcaaggaaacagcttgcctcagcaaagcctatgccaacatgtggtcactgatgtattttcacaaaagggacatgaggctactgtcattggctgtttcctcagctgttcccacctcatgggttccacaaggacgcacaacatggtcgattcatgggaaaggggagtggatgaccacggaagacatgcttgaggtgtggaacagagtatggataaccaacaacccacacatgcaggacaagacaatggtgaaaaaatggagagatgtcccttatctaaccaagagacaagacaagctgtgcggatcactgattggaatgaccaatagggccacctgggcctcccacatccatttggtcatccatcgtatccgaacgctgattggacaggagaaatacactgactacctaacagtcatggacaggtattctgtggatgctgacctgcaactgggtgagcttatctgaaacaccatctaacaggaataaccgggatacaaaccacgggtggagaaccggactccccacaacctgaaaccgggatataaaccacggctggagaaccggactccgcacttaaaatgaaacagaaaccgggataaaaactacggatggagaaccggactccacacattgagacagaagaagttgtcagcccagaaccccacacgagttttgccactgctaagctgtgaggcagtgcaggctgggacagccgacctccaggttgcgaaaaacctggtttctgggacctcccaccccagagtaaaaagaacggagcctccgctaccaccctcccacgtggtggtagaaagacggggtctagaggttagaggagaccctccagggaacaaatagtgggaccatattgacgccagggaaagaccggagtggttctctgcttttcctccagaggtctgtgagcacagtttgctcaagaataagcagacctttggatgacaaacacaaaaccact

SEQ ID NO: 9 - DNA, 10299 bp, Artificial Sequence
  Japanese encephalitis virus anyang300_ KF711994
atgactaaaaaaccaggagggcccggtaaaaaccgggctatcaatatgctgaaacgcggcctaccccgcgtactcccactagtgggagtgaagagggtagtaatgagcttgttggacggcagagggccagtacgttttgtgctggctcttatcacgttcttcaagtttacagcattagccccgaccaaggcgcttttaggccgatggaaagcagtgcaaaagagtgtggcaatgaaacatcttactagtttcaaacgagaacttggaacactcattgacgccgtgaacaagcggggcagaaagcaaaacaaaagaggaggaaatgaaggctcaatcatgtggctcgcgagcttggcagttgtcatagcttgtgcaggagcaatgaggctgtcgaatttccaggggaagcttttgatgaccattaacaacacggacgttgcagacgttatcgtgattcccacctcaaaaggagagaacagatgttgggtccgggcaatagacgtcggctacatgtgtgaggacactatcacgtacgaatgtcctaagcttaccatgggcaatgatccagaggatgtggattgctggtgtgacaaccaagaagtctacgtccaatatggacgttgcacgcggaccaggcattccaagcgaagcaggagatccgtgtcggtccaaacacatggggagagttcactagtgaataaaaaagaggcttggctggattcaacgaaagccacacgatatctcatgaaaactgagaactggatcataaggaatcctggctatgctttcctggcggcggcacttggctggatgcttggcagtaacaacggtcaacgcgtggtatttaccatcctcctgctgttggtcgctccggcttacagttttaattgtctgggaatgggcaatcgtgacttcatagaaggagccagtggagccacttgggtggacttggtgctagaaggagatagctgcttgacaatcatggcaaacgacaaaccaacattggacgtccgcatgattaacatcaaagctagccaacttgctgaggtcagaagttactgctatcatgcttcagtcactgacatctcgactgtggctcggtgccccacgactggagaagcccacaacgagaagcgagctgatagtagctatgtgtgcaaacaaggcttcactgatcgtgggtggggcaacggatgtggacttttcgggaagggaagcattgacacatgtgcaaaattctcctgcaccagcaaagcgattgggagaacaatccagccagaaaacatcaaatacgaagttggcatttttgtgcatggaaccaccacttcggaaaaccatgggaattattcagcgcaagttggggcgtcccaggcggcaaagtttacagtaacacccaatgctccttcgatgaccctcaaacttggtgactacggagaagtcacgctggactgtgagccaaggagtggactgaacactgaagcgttttacgtcatgaccgtggggtcaaggtcatttctggttcatagggaatggtttcatgacctcgctctcccctggacgtccccttcgagcacagcgtggagaaacagagaactcctcatggaatttgaagaggcgcacgccacaaaacagtccgttgtcgctcttgggtcacaggaaggaggcctccatcatgcgttggcaggagccatcgtggtggattactcaagctcagtgaagttaacatcaggccacctgaaatgtaggctgaaaatggacaaactggctctgaaaggcacaacctatggcatgtgtacagaaaaattctcgttcgcgaaaaatccggcggacactggccacggaacagttgtcattgaactctcctactctgggagtgatggcccctgcaaaattccgatcgtctccgttgcgagcctcaatgacatgacccccgttgggcggctggtgacagtgaaccctttcgtcgcgacttccagtgccaactcaaaggtgctggtcgagatggaaccccccttcggagactcctacatcgtggttgggaggggagacaagcagatcaaccaccattggcacaaagctggaagcacgctaggcaaggccttttcaacaactttgaagggagctcaaagactggcagcgttgggcgacacagcctgggactttggctctattggaggggtcttcaactccataggaaaagccgttcaccaagtgtttggtggtgccttcagaacactctttgggggaatgtcttggatcacacaagggctaatgggtgccctactactctggatgggcgtcaacgcacgagaccgatcaattgctttggccttcttagccacaggaggtgtgctcgtgttcttagcgaccaacgtgcatgctgacactggatgtgccattgacatcacaagaaaagagatgagatgtggaagtggcatctttgtgcataacgacgtggaagcctgggtggataggtataaatacttgccagaaacgcccagatccctagcgaagatcgtccacaaagcgcacaaggaaggcgtgtgcggagtcagatctgtcactagattggagcaccaaatgtgggaagccgtacgggacgaattgaacgtcctgctcaaagagaatgcagtggaccttagtgtggttgtgaacaagcccgtgggaagatatcgctcagcccccaaacgcctatccatgacgcaagagaagtttgaaatgggctggaaagcatggggaaaaagcattctctttgccccggaattggctaactccacatttgtcgtagatggacctgagacaaaggaatgccctgatgagcacagagcttggaacagcatgcaaatcgaagacttcggctttggcatcacatcaacccgtgtgtggctgaaaattagagaggagagcactgacgagtgtgatggagcgatcataggcacggctgtcaaaggacatgtggcagtccatagtgacttgtcgtactggattgagagtcgctacaacgacacatggaaacttgagagggcagtctttggagaggtcaaatcttgcacttggccagagacacacaccctttggggagatggtgttgaggaaagtgaactcatcattccgcataccatagccggaccaaaaagcaagcacaatcggagagaaggatacaagacacaaaaccagggaccttgggatgagaatggcatagtcttggactttgactattgcccagggacaaaagtcaccattacagaggactgtggcaagagaggcccttcggtcagaaccactactgacagtggaaagttgatcactgactggtgctgtcgcagttgctcccttccgcccctacgattccggacagaaaatggctgctggtacggaatggaaatcagacctgttaggcatgatgaaacaacactcgtcagatcacaggctgatgctttcaatggtgaaatggttgacccttttcagctgggccttctggtgatgtttctggccacccaggaggtccttcgcaagaggtggacggccagattgaccattcctgcggttttgggggccttacttgtgctgatgcttgggggcatcacttacactgatttggcgaggtatgtggtgctagtcgctgccgctttcgcagaggccaacggtggaggagacgtcctgcaccttgctttgattgccgtttttaagatccaaccagcatttctagtgatgaacatgcttagcacgagatggacgaaccaagaaaacgtggtcctggtcctaggggctgccttttttcaactggcctcagtagatctgcaaataggagtccacggaatcctgaatgccgccgctatagcatggatgattgtccgagcgatcaccttccccacaacctcctccgtcaccatgccagtcttagcgcttctaactccgggaatgagggctctatacctagacacttacagaatcatcctcctcgtcatagggatttgctccctgctacaagagaggaaaaagaccatggcaaaaaagaaaggagctgtactcttgggcttagcgctcacatccactggatggttctcgcccaccactatagctgccggactaatggtctgcaacccaaacaagaagagagggtggccagctactgaggttttgtcggcagttggattgatgtttgccatcgtaggtggtttggccgagttggatattgaatccatgtcaatacccttcatgctggcaggtctcatggcagtgtcctacgtggtgtcagggaaagcaacagatatgtggcttgaacgggccgccgacatcagctgggagatggatgctgcaatcacaggaagtagtcggaggctggatgtgaaactggatgatgacggagattttcacttgattgatgatcccggtgttccatggaaggtctgggtcctgcgcatgtcttgtattggcttagccgccctcacgccttgggccatcgttcccgccgccttcggttattggctcactttaaaaacaacaaaaagagggggcgtgttttgggacacgccatccccaaaaccttgctcaaaaggagacaccactacaggagtctaccgaattatggctagagggattcttggcacttaccaggccggcgtcggagtcatgtacgagaatgttttccacacactatggcacacaactagaggagcagccattatgagtggagaaggaaaattgatgccatactggggtagtgtgaaagaagaccgcatagcttacggaggcccatggaggtttgaccgaaaatggaatggaacagatgacgtgcaagtgatcgtggtagaaccggggaaggctgcagtaaacattcagacaaaaccaggagtgtttcggactcccttcggggaggttggggctgttagtctggattacccgcgaggaacatccggctcacccattctggattccaatggagatatcataggcctatacggcaatggagttgagcttggcgatggctcatacgtcagcgccatcgtgcagggtgaccgtcaggaggaaccagtcccagaagcttacaccccaaacatgttgagaaagagacagatgactgtgctagatttgcaccctggctcagggaaaaccaggaaaattctgccacaaataattaaggacgccatccagcagcgcctaagaacagctgtgctggcaccgacgcgggtggtagcagcagaaatggcagaagctttgagagggctcccagtgcgatatcaaacttcagcagtgcagagagagcaccaagggaatgaaatagtggatgtgatgtgccacgccactctgacccatagactgatgtcaccgaacagagtgcccaactacaacctatttgtcatggatgaagctcatttcactgacccagccagcatagccgcacgaggatacattgctaccaaggtggaattaggggaggcagcagccatcttcatgacagcgaccccgcctggaactacggatccttttcctgactcaaatgccccaatccatgatttgcaagatgagataccagacagggcatggagcagtggatacgaatggatcacagaatatgcgggcaaaaccgtgtggtttgtggcgagcgtaaaaatggggaatgagattgcaatgtgcctccaaagagcggggaaaaaggtcatccaactcaaccgcaagtcctatgacacagaatacccaaaatgtaagaatggagactgggattttgtcattaccaccgacatctctgaaatgggggccaacttcggtgcgagcagggtcatcgactgtagaaagagcgtgaaacccactatcttagaagagggagaaggcagagtcatcctcggaaacccatctcccataaccagtgcaagcgcagctcaacggaggggcagagtaggcagaaaccccaaccaagttggagatgaatatcactatgggggggctaccagtgaagatgacagtaacctagcccattggacagaggcaaagatcatgttagacaacatacacatgcccaatggactggtggcccagctctatggaccagagaggggaaaggctttcacaatggatggcgaataccgtctcagaggtgaagaaaagaaaaacctcttagagctgcttaggacggctgacctcccggtgtggctggcctacaaggtggcgtccaatggcattcagtacaccgacagaaagtggtgttttgatgggccgcgcacgaatgccatactggaggacaacaccgaggtagagatagtcacccggatgggtgagaggaaaatcctcaagccgagatggcttgatgcaagagtttatgcagatcaccaagccctcaagtggttcaaagactttgcagcagggaagagatcagccattagcttcatagaggtgctcggtcgcatgcctgagcatttcatgggaaagacgcgggaagctttagacaccatgtacttggttgcaacggctgagaaaggcgggaaagcacaccgaatggctctcgaagagctgccagatgcactggaaaccatcacacttattgttgccattactgcgatgacaggaggatttttcctactaatgatgcagcgaaagggtatagggaagatgggtcttggagttctagtgctcacgctagctaccttcttcctgtgggcggcagaggttcctggaaccaaaatagcagggaccctgctgatcgccctgctgctcatggtggtgctcatcccagaaccggaaaaacagaggtcacagacagataaccaactagcggtgtttctcatctgtgtcttgaccgtggttggagtggtggcagcaaacgagtacgggatgctagaaaaaaccaaagcagatctcaagagcatgtttgtcggaaagacgcaggcatcaggactgactggattgccaagcatggcactggacctgcgtccagccacagcctgggcactgtatggggggagcacagtcgtgctaacccctcttctgaagcacctgataacgtcggaatacgtcaccacatcgctagcctcaattaactcacaagctggctcattattcgtcttgccacgaggcgtaccttttaccgacctagacttgaccgttggccttgtcttccttggctgttggggtcaaatcaccctcacaacgtttctgacagccatgtttctggcgacacttcattatgggtacatgctccctggatggcaagcagaagcactcagggctgcccagagaaggacagcggctggaataatgaagaatgccgttgttgacggaatggtcgccactgatgtgcctgaactggaaaggactacccctctgatgcaaaagaaagtcggacaggtgctcctcataggggtaagcgtagcagcgttcctcgtcaaccctaatgtcaccactgtgagagaagcaggagtattggtgacggcggctacgctcactttgtgggacaatggagccagtgccgtttggaattccaccacagccacgggactctgccatgttatgcgaggtagctacctggctggaggctccattgcttggactctcatcaagaacgctgataagccctccttgaaaaggggaaggcctgggggcaggacgctaggggagcaatggaaggaaaaactaaatgccatgagcagagaagagttttttaaataccgaagagaggccataatcgaggtggaccgcactgaagcacgcagggctagacgtgaaaataacatagtgggaggacatccggtttcgcgaggctcagcaaaactccgttggctcgtggagaaaggatttgtctcgccaataggaaaagtcattgatctagggtgtgggcgtggaggatggagctactacgcagcaaccctgaagaaggtccaggaagtcagaggatacacgaaaggtggggcgggacatgaagaaccgatgctcatgcagagctacggctggaacctggtctccttgaagagtggagtggatgtgttttacaaaccttcagaacccagtgacaccctgttctgtgacataggggaatcctctccaagtccagaagtagaagaacaacgcacactacgcgtcctagagatgacatctgactggttgcaccgaggacctagagagttctgcataaaagttctctgcccttacatgcccaaggttatagaaaaaatggaagttctgcagcgccgcttcggaggtgggctattgcgtctccccctgtcccgaaactccaatcacgagatgtattgggttagtggggccgctggcaatgtggtgcacgctgtgaacatgaccagccaggtgctactggggcgaatggatcgcacagtgtggagagggccaaagtatgaggaagatgtcaacctagggagcggaacaagagccgtgggaaagggagaagtccatagcaatcaggagaaaatcaagaagagaatccagaagcttaaagaagaattcgccacaacgtggcacaaagaccctgagcatccataccgcacttggacataccacggaagctatgaagtgaaggctactggctcagccagctctctcgtcaacggagtggtgaagctcatgagcaaaccttgggacgccattgccaacgtcaccaccatggccatgactgacaccaccccttttggacagcaaagagttttcaaggagaaagttgacacgaaggctcctgagccaccagctggcgccaaagaagtgctcaacgagaccaccaactggctgtgggcccacttgtcacgggaaaaaagaccccgcttgtgcaccaaggaagaatttataaagaaagtcaacagcaacgcggctcttggagcagtgttcgctgaacagaatcaatggagcacggctcgtgaggctgtggatgacccgcggttttgggagatggttgatgaagaaagggaaaaccatctgcgaggagagtgtcacacatgtatctacaatatgatggggaaaagagagaagaaacctggagagtttggaaaagctaaaggaagcagggccatttggttcatgtggcttggagcacggtatctagagtttgaagctttggggttcctgaatgaagaccattggctgagccgagagaattcaggaggtggagtggaaggctcaggcgtccaaaagctgggatacatcctccgtgacatagcaggaaagcaaggagggaaaatgtacgctgatgacaccgccggatgggacactagaattaccagaactgatttagaaaatgaagctaaggtgctggagctcctagacggtgaacaccgcatgctcgcccgagccataattgaactgacttacaggcacaaagtggtcaaggtcatgagacctgcagcagaaggaaagaccgtaatggacgtgatatcaagagaagatcaaagggggagtggacaggtggtcacttatgcccttaacacttttacgaacatcgctgtccagctcgtcaggttgatggaggctgagggggtcattggaccacaacacttggaacagctacctagaaaaaccaagatagctgtcaggacctggctctttgagaatggagaggagagagtgaccaggatggcgatcagcggagacgactgtgtcgtcaagccgctggacgacagattcgccacagccctccacttcctcaacgcaatgtcaaaggtcagaaaagacatccaggaatggaagccttcgcatggctggcacgactggcagcaagttcccttctgctctaaccattttcaggagattgtgatgaaagatggaaggagtatagttgtcccgtgcagaggacaggatgagctgataggcagggctcgcatctctccaggagctggatggaatgtgaaggacacagcttgcctggccaaagcatatgcacagatgtggctactcctatacttccatcgtagggacttgcgtctcatggcaaatgcgatttgctcagcagtgccagtggattgggtgcccacaggcaggacgtcctggtcaatacactcgaaaggagagtggatgaccacggaagacatgctgcaggtctggaacagagtctggattgaagaaaatgaatggatgatggacaagactccaatcacaagctggacagacgttccgtatgtgggaaagcgtgaggacatctggtgtggtagcctcatcggaacgcgatccagagcaacctgggctgagaacatctatgcggcgataaaccaggttagagctgtcattgggaaagaaaattatgttgactacatgacctcactcaggagatacgaagacgtcttcattcaggaagacagggtcatctag

SEQ ID NO: 10 - DNA, 10966 bp, Artificial Sequence
  West Nile virus_ KT359349
tttgtgaggattaacaacaattaacacagtgcgagctgtttcttagcacgaagatctcgatgtctaagaaaccaggagggcccggtaaaaaccgggctgtcaatatgctaaaacgcggtatgccccgcggattgtccttgataggactgaagagggctatgctgagtctgattgacgggaaaggcccaatacgtttcgtgttggctcttttggcgtttttcagattcactgcaattgctccgactcgtgcggtgctggacagatggagaggcgtcaacaaacaaacagcgatgaagcatctcttgagtttcaagaaagaactaggaactctgaccagtgccatcaaccgccggagcacaaaacaaaagaaaagaggaggcacagcaggctttactatcttgcttgggctgatcgcttgtgctggagctgtgaccctctcgaacttccagggcaaagtgatgatgacagtcaatgcaaccgatgtcactgacgtgattaccatcccaacagctgctgggaaaaacctgtgcattgtgagggctatggacgtgggatacctttgtgaggatactatcacttatgaatgtccggtcctagctgctggaaatgaccctgaagacattgactgctggtgcacgaaatcatctgtttacgtgcgctatggaagatgcacaaaaactcggcattcccgtcgaagcagaaggtctctgactgtccagacacatggagaaagtacactggccaacaagaaaggagcttggttggacagcacaaaagccacgagatatctggtgaagacagaatcatggatactgagaaacccgggctatgccctcgttgcagcggtcattggatggatgctgggaagcaacacaatgcaacgcgtcgtgtttgccatcctattgctcctggtggcaccagcatacagctttaattgcttgggaatgagtaacagagacttcctggagggagtgtctggagccacatgggttgatctggtactggaaggcgatagttgtgtgaccataatgtcaaaggacaagccaaccattgatgtcaaaatgatgaacatggaagcagccaacctcgcagatgtgcgcagctactgttacctagcttcggtcagtgacttgtcaacgagagccgcgtgtccaaccatgggtgaagcccacaacgagaaaagagctgaccccgccttcgtttgcaagcaaggcgttgtggacagaggatggggaaatggctgcggactgtttggaaagggaagcattgacacatgcgcgaagtttgcctgtacaaccaaagcaactggatggatcatccagaaggagaacatcaagtatgaggtcgccatatttgtgcatggcccgacgactgttgaatctcatggcaattattcaacacagatggaggccacccaggctggaagattcagtataactccatcggcgccatcttacacgctaaagttgggtgagtatggtgaggtcacggttgactgtgagccacggtcaggaatagacactagcgcctattacgttatgtcagttggtgcgaagtccttcctggttcaccgagaatggtttatggatctgaacctgccatggagcagtgctggaagcaccacatggaggaatcgggaaacactgatggagtttgaagaacctcatgccaccaaacaatctgttgtggctctagggtcgcaggaaggtgcattgcaccaagctctggccggagcgattcctgttgagttctcaagcaatactgtgaagttgacttcaggacatctgaagtgtagggtgaagatggagaagttgcagctgaagggaacaacatatggagtatgttcaaaagcgtttaaattcgctgggactcccgctgacactggccatggaacggtggtgttggaactgcaatacaccggaacagacggtccctgcaaagtgcccatttcttccgtagcttccctgaatgacctcacacctgttggaagactggtgaccgtgaatccatttgtgtctgtggccacggctaactcgaaggtcttgattgaactcgaacccccgtttggtgactcttacatcgtggtaggaagaggagaacagcagataaaccaccactggcacaaatctgggagcagcatcggaaaggcctttaccactacactcagaggagctcaacgactcgcagctcttggagacactgcttgggattttgggtcagttggaggggttttcacctcagtggggaaagccatacaccaagtctttggaggagcttttagatcactctttggagggatgtcctggatcacacagggacttctaggagcccttctgttgtggatgggaatcaatgcccgtgacaggtcaattgccatgacgtttcttgcggttggaggagttttgctcttcctttcggtcaacgtccatgctgacacaggctgtgccattgatattggcaggcaagagctccggtgtggaagtggagtgtttatccacaacgatgtggaagcctggatggatcgttacaagttctacccggagacaccacaaggcctagcaagaattattcagaaagcacatacagaaggagtctgcggcttgcgttccgtttccagactcgagcaccaaatgtgggaagccattaaggatgagctgaacaccctgttgaaagagaatggagtcgacttgagtgtcgtggtggaaaaccaaaatgggatgtataaagcagcaccaaaacgtttggctgccaccaccgaaaaactggagatgggttggaaggcttggggcaagagcatcatctttgctccagaactagctaacaacacctttgtcatcgacggtcctgagactgaggaatgcccaacggccaaccgagcatggaacagcatggaggtagaagactttggatttggattgacaagcactcgcatgttcctgaggattcgggaaacgaacacaactgaatgcgactcgaagatcataggaaccgccgtcaagaacaacatggctgtgcacagtgatctgtcgtactggatagagagcggactcaacgacacctggaagcttgagagggcggttctaggagaagtcaaatcatgcacctggccagaaacccacactttgtggggtgatggagttctggaaagtgatctcatcatacccatcaccttggcaggacccagaagcaatcataacaggagaccagggtacaaaactcagaaccaaggtccatgggatgaggggcgtgtcgagattgactttgactattgcccaggaacaacagtaactataagtgatagttgcggacaccgtggacctgcggcacgcacaaccactgagagtgggaagctcattacagactggtgctgcagaagctgcaccctccctccactgcgcttccagactgagaatggctgttggtatggaatggaaattcgacccacgcggcacgacgaaaagaccctcgtgcaatcgagagtgaatgcatacaacgccgacatgattgatccttttcagttgggccttctggtcgtgttcttggccacccaggaggtccttcgcaagaggtggacggccaagatcagcattccagctatcatgcttgcactcctagtcctagtgtttgggggtattacgtacactgatgtcctgcgatatgtcattctcgtcggcgccgcgtttgctgaagcaaactcaggaggagacgttgtgcacttggcactcatggctacattcaagattcaaccagtctttctggtggcttcctttttgaaggcaaggtggaccaaccaagagagtattttgctcatgcttgcagctgctttctttcaaatggcttactatgacgccaagaatgttttgtcatgggaagtgcctgacgttttgaactctctctccgttgcgtggatgattctcagagctataagcttcaccaacacttcaaatgtggtggtgccgctgctggcccttctaacacctggactaaaatgcctaaaccttgacgtgtacagaattttgctactcatggttggagttggaagcctcatcaaagaaaaaaggagctctgcagcaaaaaagaaaggggcttgcctcatctgcctagcgctggcgtctacaggagtgttcaatccaatgatacttgcagctgggctgatggcttgcgaccccaaccgcaagcggggctggcctgccacagaagtgatgactgcagttggactcatgtttgccatcgttgggggtctggcagaacttgatatagactctatggctatccccatgaccattgccggactcatgttcgtggcatttgtcatctctggaaagtcaacagacatgtggattgagaggacggctgatattacttgggagagtgacgctgaaatcacaggctctagtgaaagagtagatgttaggctggatgatgatggaaattttcaattgataaatgaccccggggcgccatggaaaatttggatgcttaggatggcctgcctggcaataagtgcctacacaccttgggcgattcttccctcggtcattggattctggataacccttcagtacacaaagagaggaggtgtcctttgggacacaccatcacccagggagtacaagaagggtgataccaccactggcgtttacagaatcatgactcgaggtctgcttggcagttaccaagctggagccggagtgatggtagagggagtgttccacacactatggcacaccactaagggagctgctctcatgagtggtgaaggacgtctggatccctattgggggagcgtgaaagaagaccggctttgctatggggggccatggaaactccaacataaatggaatggacatgatgaggtccaaatgattgttgtggagccaggaaaaaatgtgaaaaacgtccagactaagcccggagtgtttaagacaccagaaggagaaattggggcagttacgctagactatcccactggaacgtcaggttcccccattgtggataaaaatggagatgtgattggattgtatgggaacggcgtcatcatgcctaatggttcatacataagcgccattgtgcaaggagagagaatggaagaaccggcaccagctggcttcgaacctgaaatgttgaggaagaaacagatcactgtccttgatctgcaccccggagcaggaaagacgcgcaagatacttccccaaatcatcaaggaggccatcaacaaaagattgaggacggctgtactggcacccaccagggtcgttgctgctgagatgtctgaggccctgagaggacttcccatccggtatcaaacctcagcagtgcacagagagcacagtggaaatgagatcgttgatgtcatgtgccatgccactctcacacacaggctgatgtctccacacagagtccccaattacaatctgttcataatggatgaagcccatttcacggatccagcgagcatcgcagccagaggatacatagcaaccaaggttgaattgggcgaagccgccgcgattttcatgacggcaacgccacccgggacttctgacccctttccagagtctaatgctcctatctcggacatgcaaacagagatcccagacagagcctggaacactggatatgaatggataactgagtatgttggaaagaccgtttggtttgttccaagtgtgaaaatgggaaatgagattgccctctgtctgcaacgggcggggaagaaggttattcagctgaacagaaagtcctacgagacagagtaccctaagtgcaagaacgatgattgggattttgtcatcaccacagacatatcagaaatgggagcaaacttcaaggcaagcagagtgatcgacagccgcaaaagcgtgaaacccaccatcattgaggaaggtgatggaagagtcatcctgggggaaccctcagccatcacggctgccagcgctgctcagcggagaggacgcataggaagaaacccatcacaagttggtgatgagtattgctatggagggcacacaaatgaggatgattccaactttgcccactggacagaggctcgcatcatgctagacaacatcaacatgccgaatggtctggtggcccaactatatcagcctgagcgcgagaaggtgtacaccatggacggggaatataggctcagaggggaagaacggaagaacttccttgaattcctgagaacagctgatttaccagtctggctcgcttacaaagtggcagcagcgggaatatcataccatgaccggaagtggtgctttgatggacctcgaaccaacacgattcttgaagacaacaatgaagttgaagtcatcacgaagttgggtgagagaaagatcctaagacccaggtgggcggatgccagagtgtactcagaccaccaagctctaaagtccttcaaagactttgcatcagggaaacgatcacaaatcgggctcgttgaggtgctcgggagaatgcctgagcacttcatggggaaaacttgggaggcgttggacacgatgtatgtggtggcaaccgctgaaaaaggaggtcgagctcacaggatggctcttgaggagctaccggacgcccttcagacaatagctttgattgcactattgagtgtgatgtccttgggtgtgttttttctactcatgcaaaggaaaggcattggtaagattggcttgggaggagtgatcttaggagctgccacattcttctgctggatggctgaagtcccaggaacgaaaatagcaggcatgctcctgctttccctgctgctcatgattgttttgattccggagccggaaaagcagcgctcacagactgacaaccagcttgccgtgttcttgatttgtgtgctcacactggtcagcgccgtggctgccaatgaaatgggttggctggacaagaccaagaatgacattagcagcctgttgggacacaagccagaaactagagagacgaccctgggagttgagaactttttgcttgatctgcggccggctacagcatggtcgctctatgccgtaacgacagccgttcttacccctctgctgaaacatctaattacgtcagactacatcaacacttcgctgacctcaataaacgtccaagccagtgcgttgttcaccttggccagaggcttcccttttgtggacgttggtgtgtcagctctcttgctagcggccgggtgctggggccaagtgaccctgactgtgactgtgactgcagctgccctgctcttttgccactatgcttacatggtaccaggctggcaagcggaagccatgcgatccgcccagcggcggacagctgctggcatcatgaaaaatgcagtggtggatgggatcgtggctactgatgtacctgaacttgagcgaacaactccagtcatgcagaaaaaagttggacagatcatgctgatcttggtgtcaatggccgcggttgtcgtcaatccatcagtgagaactgtcagagaggctggaattctgaccacagcagcagcagtcaccttatgggagaatggtgctagttcagtgtggaatgcaacgacagctattgggctttgtcacatcatgcgaggaggatggctctcgtgtctctccatcacgtggactctcatcaaaaacatggagaaaccaggcctcaagaggggtggagccaagggacgcacgctaggggaagtttggaaggagagactcaaccacatgacgaaggaagaatttaccagatacagaaaagaagccatcactgaagtcgaccgctccgcggcaaaacatgccaggagagagggaaacatcactggaggccatccagtctcacggggaaccgcgaaattacggtggttagtggaaaggcgtttcctcgagccagtgggaaaggttgtggatctcggatgtggtaggggcggctggtgttattacatggctacccagaagagggtacaggaagtgaaagggtacacgaaaggaggacctggccatgaagagccacaactggtgcagagctatggttggaatattgttaccatgaagagtggagtcgacgtcttctacagaccatcagaagcgagcgacacactgctctgtgacattggagagtcatcgtcaagtgccgaggtagaagaacaccgcaccgtccgtgtcttggagatggtggaagactggctgcacagaggacctaaggaattctgcatcaaagtgctatgcccttacatgcccagagtgattgagaagatggaaacactccaaaggcgatatggaggtggccttgtgagaaaccccctttcacgcaactctacccatgagatgtactgggtgagccacgcttcaggcaacattgtccactccgtgaacatgacaagccaggtgcttctggggaggatggaaaagaaaacatggaagggaccccagtttgaggaagatgtcaacttgggaagtggaacgcgggcagtagggaagcctctcctcaattctgatactagcaagatcaagaaccgaattgagaggctgaagaaagaatacagctccacatggcaccaggatgcgaatcacccctacaggacctggaactaccacggaagctatgaagtgaaaccaaccggctcagccagctcccttgtgaatggggtagttagattactctcaaaaccatgggacactatcaccaatgtgaccacgatggccatgacagacaccactcctttcggtcaacaacgagtgttcaaggaaaaggtggatacaaaggctccagagcctccagaaggggtcaaatacgtcctcaatgagaccacgaactggttgtgggcttttctagcccgcgataagaaacccaggatgtgttcccgggaggaattcattggaaaagtcaacagtaatgccgccctaggagcgatgtttgaagaacagaaccaatggaagaacgcccgggaagccgtggaggatccaaagttttgggagatggtggatgaggagcgtgaggcgcatctccgtggagaatgcaacacctgcatctacaacatgatgggaaagagagagaagaagcctggagagttcggcaaagctaaaggcagcagagccatttggttcatgtggctaggggcccgcttcctggagtttgaagctctcggattcctcaatgaagaccactggctgggtaggaagaactcaggaggaggagttgaaggcttaggactgcagaagcttgggtacatcttgaaggaagtcggaacaaagcctggaggaaagatctacgccgatgataccgcaggctgggacacacgcatcaccaaagctgacctcgagaacgaagcgaaggttcttgaactgctggacggagaacaccgacgcctagcgcggtccatcattgagctcacataccgacacaaagtcgtgaaagtgatgaggccagcggccgacgggaaaactgtgatggacgtcatctccagagaggatcagagaggaagcgggcaggtagtgacttacgccctgaacaccttcactaatctagcagttcagctggtcagaatgatggagggggagggggtcattggacctgacgatgttgaaaaactgggaaaaggaaaaggccctaaggtcagaacctggctgtttgagaatggcgaggagcgtctcagtcgcatggccgtcagcggtgatgactgcgtggtgaaacctttggacgaccgcttcgccacatcactacacttcctaaatgccatgtcaaaggtccgcaaagacatccaggaatggaaaccctcgacagggtggtatgactggcagcaggtcccattctgttcaaaccatttcacggaactgatcatgaaggacggcaggacgttggtggtcccgtgtcgtggacaagacgagttgattggacgggccagaatctctccaggggctggatggaatgtgcgcgacaccgcctgcctggcgaagtcatacgcgcagatgtggctgttgctttattttcaccgtagagacctgagattgatggctaacgccatctgttccgctgtgcctgtcaactgggttcccacagggcgtaccacctggtcgatccacgcaaaaggagaatggatgacgacagaagacatgctcgcagtctggaacagagtgtggattgaggagaatgagtggatggaagacaaaacaccagttgagaggtggagtgatgttccatactccggaaagagagaagacatttggtgtggcagtttgattggcacacgaacccgcgctacttgggctgaaaatatccatgtggcaatcaatcaggtccgttcggtgattggagaagagaagtatgtggattacatgagctccctgaggaggtatgaagacaccattgtagttgaggacactgttttgtaaataataaagctgtattgagtagttgtatagttgtagtgtttatagcaatttgaattatgattaattatttaggcttaagatagcattatagttagtttagtgtgaataggttttattgagaatggaagtcaggccagattaatgctgccaccggaagttgagtagacggtgctgcctgcggctcaaccccaggaggactgggtgaccaaagctgcgaggtgatccacgtaagccctcagaaccgtctcggaaggaggaccccacgtgctttagcctcaaagcccagtgtcagaccacactctagtgtgccactctgcggagagtgcagtctgcgatagtgccccaggtggactgggttaacaaaggcaaaacatcgccccacgcggccataaccctggctatggtgttaaccagggagaagggactagaggttagaggagaccccgcgtcaaaaagtgcacggcccaacatggctgaagctgtaagccaagggaaggactagaggttagaggagaccccgtgccaataacaccaaaagaaacagcatattgacacctgggatagactaggggatcttctgctctgcacaaccagccacacgg

SEQ ID NO: 11 - DNA, 45 bp, Artificial Sequence
  5' end
taatacgactcactatagggtttgctagttattgctcagcggtgg

SEQ ID NO: 12 - DNA, 45 bp, Artificial Sequence
  3' end
ccaccgctgagcaataactagctttccctatagtgagtcgtatta

SEQ ID NO: 13 - DNA, 26 bp, Artificial Sequence
  FL-F1
gccatatggtacatgtggctgggagc

SEQ ID NO: 14 - DNA, 32 bp, Artificial Sequence
  FL-R3
gtkattcttgtgtcccawccggctgtgtcatc

SEQ ID NO: 15 - DNA, 32 bp, Artificial Sequence
  FL-R4
gtgatgcgrgtgtcccagccrgckgtgtcatc

SEQ ID NO: 16 - DNA, 406 bp, Artificial Sequence
  Panel(KT359349|West Nile virus2|2014/hun_ex)
taatacgactcactatagggtttgctagttattgctcagcggtgggtggagaatgcaacacctgcatctacaacatgatgggaaagagagagaagaagcctggagagttcggcaaagctaaaggcagcagagccatttggttcatgtggctaggggcccgcttcctggagtttgaagctctcggattcctcaatgaagaccactggctgggtaggaagaactcaggaggaggagttgaaggcttaggactgcagaagcttgggtacatcttgaaggaagtcggaacaaagcctggaggaaagatctacgccgatgataccgcaggctgggacacacgcatcaccaaagctgacctcgagaaccaccgctgagcaataactagctttccctatagtgagtcgtatta